European Patent Specification EP 3 248 610 B1, published December 20, 2023. Title: FGF21 Mutants and Uses Thereof. Applicant: Amgen, Inc. Application not yet assigned. The sequence listing filed with the application follows.

SEQUENCE LISTING (165 sequences)

SEQ ID NO: 1 - DNA, 630 bp, Homo sapiens
  CDS (1)..(630)
atggactcggacgagaccgggttcgagcactcaggactgtgggtttctgtgctggctggtcttctgctgggagcctgccaggcacaccccatccctgactccagtcctctcctgcaattcgggggccaagtccggcagcggtacctctacacagatgatgcccagcagacagaagcccacctggagatcagggaggatgggacggtggggggcgctgctgaccagagccccgaaagtctcctgcagctgaaagccttgaagccgggagttattcaaatcttgggagtcaagacatccaggttcctgtgccagcggccagatggggccctgtatggatcgctccactttgaccctgaggcctgcagcttccgggagctgcttcttgaggacggatacaatgtttaccagtccgaagcccacggcctcccgctgcacctgccagggaacaagtccccacaccgggaccctgcaccccgaggaccagctcgcttcctgccactaccaggcctgccccccgcacccccggagccacccggaatcctggccccccagccccccgatgtgggctcctcggaccctctgagcatggtgggaccttcccagggccgaagccccagctacgcttcctga

SEQ ID NO: 2 - protein, 209 aa, Homo sapiens [sequence omitted]

SEQ ID NO: 3 - DNA, 546 bp, Homo sapiens
  CDS (1)..(546)
caccccatccctgactccagtcctctcctgcaattcgggggccaagtccggcagcggtacctctacacagatgatgcccagcagacagaagcccacctggagatcagggaggatgggacggtggggggcgctgctgaccagagccccgaaagtctcctgcagctgaaagccttgaagccgggagttattcaaatcttgggagtcaagacatccaggttcctgtgccagcggccagatggggccctgtatggatcgctccactttgaccctgaggcctgcagcttccgggagctgcttcttgaggacggatacaatgtttaccagtccgaagcccacggcctcccgctgcacctgccagggaacaagtccccacaccgggaccctgcaccccgaggaccagctcgcttcctgccactaccaggcctgccccccgcacccccggagccacccggaatcctggccccccagccccccgatgtgggctcctcggaccctctgagcatggtgggaccttcccagggccgaagccccagctacgcttcctga

SEQ ID NO: 4 - protein, 181 aa, Homo sapiens
HPIPDSSPLLQFGGQVRQRYLYTDDAQQTEAHLEIREDGTVGGAADQSPESLLQLKALKPGVIQILGVKTSRFLCQRPDGALYGSLHFDPEACSFRELLLEDGYNVYQSEAHGLPLHLPGNKSPHRDPAPRGPARFLPLPGLPPAPPEPPGILAPQPPDVGSSDPLSMVGPSQGRSPSYAS

SEQ ID NO: 5 - DNA, 630 bp, Homo sapiens
  CDS (1)..(630)
atggactcggacgagaccgggttcgagcactcaggactgtgggtttctgtgctggctggtcttctgctgggagcctgccaggcacaccccatccctgactccagtcctctcctgcaattcgggggccaagtccggcagcggtacctctacacagatgatgcccagcagacagaagcccacctggagatcagggaggatgggacggtggggggcgctgctgaccagagccccgaaagtctcctgcagctgaaagccttgaagccgggagttattcaaatcttgggagtcaagacatccaggttcctgtgccagcggccagatggggccctgtatggatcgctccactttgaccctgaggcctgcagcttccgggagctgcttcttgaggacggatacaatgtttaccagtccgaagcccacggcctcccgctgcacctgccagggaacaagtccccacaccgggaccctgcaccccgaggaccagctcgcttcctgccactaccaggcctgccccccgcactcccggagccacccggaatcctggccccccagccccccgatgtgggctcctcggaccctctgagcatggtgggaccttcccagggccgaagccccagctacgcttcctga

SEQ ID NO: 6 - protein, 209 aa, Homo sapiens
MDSDETGFEHSGLWVSVLAGLLLGACQAHPIPDSSPLLQFGGQVRQRYLYTDDAQQTEAHLEIREDGTVGGAADQSPESLLQLKALKPGVIQILGVKTSRFLCQRPDGALYGSLHFDPEACSFRELLLEDGYNVYQSEAHGLPLHLPGNKSPHRDPAPRGPARFLPLPGLPPALPEPPGILAPQPPDVGSSDPLSMVGPSQGRSPSYAS

SEQ ID NO: 7 - DNA, 546 bp, Homo sapiens
  CDS (1)..(546)
caccccatccctgactccagtcctctcctgcaattcgggggccaagtccggcagcggtacctctacacagatgatgcccagcagacagaagcccacctggagatcagggaggatgggacggtggggggcgctgctgaccagagccccgaaagtctcctgcagctgaaagccttgaagccgggagttattcaaatcttgggagtcaagacatccaggttcctgtgccagcggccagatggggccctgtatggatcgctccactttgaccctgaggcctgcagcttccgggagctgcttcttgaggacggatacaatgtttaccagtccgaagcccacggcctcccgctgcacctgccagggaacaagtccccacaccgggaccctgcaccccgaggaccagctcgcttcctgccactaccaggcctgccccccgcactcccggagccacccggaatcctggccccccagccccccgatgtgggctcctcggaccctctgagcatggtgggaccttcccagggccgaagccccagctacgcttcctga

SEQ ID NO: 8 - protein, 181 aa, Homo sapiens
HPIPDSSPLLQFGGQVRQRYLYTDDAQQTEAHLEIREDGTVGGAADQSPESLLQLKALKPGVIQILGVKTSRFLCQRPDGALYGSLHFDPEACSFRELLLEDGYNVYQSEAHGLPLHLPGNKSPHRDPAPRGPARFLPLPGLPPALPEPPGILAPQPPDVGSSDPLSMVGPSQGRSPSYAS

SEQ ID NO: 9 - protein, 10 aa, Artificial Sequence
  portion of a mature human FGF21 polypeptide
MHPIPDSSPL

SEQ ID NO: 10 - DNA, 681 bp, Homo sapiens
  CDS (1)..(681)
gacaaaactcacacatgtccaccttgtccagctccggaactcctggggggaccgtcagtcttcctcttccccccaaaacccaaggacaccctcatgatctcccgtacccctgaggtcacatgcgtggtggtggacgtgagccacgaagaccctgaggtcaagttcaactggtacgtggacggcgtggaggtgcataatgccaagacaaagccgcgtgaggagcagtacaacagcacgtaccgtgtggtcagcgtcctcaccgtcctgcaccaggactggctgaatggcaaggagtacaagtgcaaggtctccaacaaagccctcccagcccccatcgagaaaaccatctccaaagccaaagggcagccccgagaaccacaggtgtacaccctgcccccatcccgtgatgagctgaccaagaaccaggtcagcctgacctgcctggtcaaaggcttctatcccagcgacatcgccgtggagtgggagagcaatgggcagccggagaacaactacaagaccacgcctcccgtgctggactccgacggctccttcttcctctacagcaagctcaccgtggacaagagccgttggcagcaggggaacgtcttctcatgctccgtgatgcatgaggctctgcacaaccactacacgcagaagagcctctccctgtctccgggtaaa

SEQ ID NO: 11 - protein, 227 aa, Homo sapiens
DKTHTCPPCPAPELLGGPSVFLFPPKPKDTLMISRTPEVTCVVVDVSHEDPEVKFNWYVDGVEVHNAKTKPREEQYNSTYRVVSVLTVLHQDWLNGKEYKCKVSNKALPAPIEKTISKAKGQPREPQVYTLPPSRDELTKNQVSLTCLVKGFYPSDIAVEWESNGQPENNYKTTPPVLDSDGSFFLYSKLTVDKSRWQQGNVFSCSVMHEALHNHYTQKSLSLSPGK

SEQ ID NO: 12 - DNA, 40 bp, Artificial Sequence
  PCR primer
aggaggaataacatatgcatccaattccagattcttctcc

SEQ ID NO: 13 - DNA, 33 bp, Artificial Sequence
  PCR primer
tagtgagctcgaattcttaggaagcgtagctgg

SEQ ID NO: 14 - DNA, 41 bp, Artificial Sequence
  PCR primer
ggagatatacatatgccaattccagattcttctccattatt

SEQ ID NO: 15 - DNA, 34 bp, Artificial Sequence
  PCR primer
catatgtatatctccttcttaaagttaaacaaaa

SEQ ID NO: 16 - DNA, 34 bp, Artificial
  PCR primer
aaaacaaattgaaattcttcctctatatgtatac

SEQ ID NO: 17 - DNA, 63 bp, Artificial Sequence
  sense strand from a portion of an FGF21 expression construct
ttttgtttaactttaagaaggagatatacatatgcatccaattccagattcttctccattatt

SEQ ID NO: 18 - DNA, 63 bp, Artificial
  antisense strand from a portion of an FGF21 expression construct
aaaacaaattgaaattcttcctctatatgtatacgtaggttaaggtctaagaagaggtaataa

SEQ ID NO: 19 - DNA, 34 bp, Artificial Sequence
  PCR primer
aggaggaataacatatggacaaaactcacacatg

SEQ ID NO: 20 - DNA, 23 bp, Artificial Sequence
  PCR primer
ggatccaccaccaccgctaccac

SEQ ID NO: 21 - DNA, 39 bp, Artificial Sequence
  PCR primer
ggtggtggtggatcccatccaattccagattcttctcca

SEQ ID NO: 22 - DNA, 33 bp, Artificial Sequence; identical to SEQ ID NO: 13
  PCR primer

SEQ ID NO: 23 - DNA, 27 bp, Artificial Sequence
  PCR primer
atggtggaaccttcccagggccgaagc

SEQ ID NO: 24 - DNA, 30 bp, Artificial Sequence
  PCR primer
ggaaggttccaccatgctcagagggtccga

SEQ ID NO: 25 - DNA, 50 bp, Artificial Sequence
  sense strand from a portion of an FGF21 expression construct
ctcctcggaccctctgagcatggtgggaccttcccagggccgaagcccca

SEQ ID NO: 26 - DNA, 30 bp, Artificial
  PCR primer
agcctgggagactcgtaccaccttggaagg

SEQ ID NO: 27 - DNA, 50 bp, artificial
  antisense strand from a portion of an FGF21 expression construct
gaggagcctgggagactcgtaccaccctggaagggtcccggcttcggggt

SEQ ID NO: 28 - protein, 15 aa, Artificial Sequence
  G5SG3SG4S (L15) Linker
GGGGGSGGGSGGGGS

SEQ ID NO: 29 - protein, 4 aa, Artificial
  G4 Linker
GGGG

SEQ ID NO: 30 - protein, 5 aa, Artificial
  G5 Linker
GGGGG

SEQ ID NO: 31 - protein, 15 aa, Artificial
  (G4S)3 Linker
GGGGSGGGGSGGGGS

SEQ ID NO: 32 - protein, 8 aa, Artificial
  G3KG4 linker
GGGKGGGG

SEQ ID NO: 33 - protein, 8 aa, Artificial
  G3NGSG2 Linker
GGGNGSGG

SEQ ID NO: 34 - protein, 8 aa, Artificial
  G3CG4 linker
GGGCGGGG

SEQ ID NO: 35 - protein, 5 aa, Artificial
  GPNG2 Linker
GPNGG

SEQ ID NO: 36 - DNA, 549 bp, Artificial Sequence
  FGF21 RG
  CDS (1)..(549)
atgcatccaattccagattcttctccattattacaattcgggggccaagtccggcagcgttacctctacacagatgatgcccagcagacagaagcccacctggagatcagggaggacgggacggtggggggtgctgctgaccagagccccgaaagtctcctgcagctgaaagccttgaagccgggtgttattcaaatcttgggtgtcaagacatccaggttcctgtgccagcggccagatggggccctgtatggatcgctccactttgaccctgaggcctgcagcttccgtgagcgtcttcttgaggacggttacaatgtttaccagtccgaagcccacggcctcccgctgcacctgccagggaacaagtccccacaccgtgaccctgcaccccgaggaccagctcgcttcctgccactaccaggcctgccccccgcacccccggagccacccggaatcctggccccccagccccccgatgtgggctcctcggaccctctgagcatggtgggtggttcccagggccgaagccccagctacgcttcctaa

SEQ ID NO: 37 - protein, 182 aa, Artificial Sequence
  Synthetic Construct
MHPIPDSSPLLQFGGQVRQRYLYTDDAQQTEAHLEIREDGTVGGAADQSPESLLQLKALKPGVIQILGVKTSRFLCQRPDGALYGSLHFDPEACSFRERLLEDGYNVYQSEAHGLPLHLPGNKSPHRDPAPRGPARFLPLPGLPPAPPEPPGILAPQPPDVGSSDPLSMVGGSQGRSPSYAS

SEQ ID NO: 38 - DNA, 546 bp, Artificial Sequence
  FGF21 RGE
  CDS (1)..(546)
catccaattccagattcttctccattattacaattcgggggccaagtccggcagcgttacctctacacagatgatgcccagcagacagaagcccacctggagatcagggaggacgggacggtggggggtgctgctgaccagagccccgaaagtctcctgcagctgaaagccttgaagccgggtgttattcaaatcttgggtgtcaagacatccaggttcctgtgccagcggccagatggggccctgtatggatcgctccactttgaccctgaggcctgcagcttccgtgagcgtcttcttgaggacggttacaatgtttaccagtccgaagcccacggcctcccgctgcacctgccagggaacaagtccccacaccgtgaccctgcaccccgaggaccagctcgcttcctgccactaccaggcctgccccccgcacccccggagccacccggaatcctggccccccagccccccgatgtgggctcctcggaccctctgagcatggtgggtggttcccagggccgaagccccagctacgaatcctaa

SEQ ID NO: 39 - protein, 181 aa, Artificial Sequence
  Synthetic Construct
HPIPDSSPLLQFGGQVRQRYLYTDDAQQTEAHLEIREDGTVGGAADQSPESLLQLKALKPGVIQILGVKTSRFLCQRPDGALYGSLHFDPEACSFRERLLEDGYNVYQSEAHGLPLHLPGNKSPHRDPAPRGPARFLPLPGLPPAPPEPPGILAPQPPDVGSSDPLSMVGGSQGRSPSYES

SEQ ID NO: 40 - DNA, 1272 bp, Artificial Sequence
  WT21-L15-Fc
  CDS (1)..(1272)
atgcatccaattccagattcttctccattattacaattcgggggccaagtccggcagcggtacctctacacagatgatgcccagcagacagaagcccacctggagatcagggaggatgggacggtggggggcgctgctgaccagagccccgaaagtctcctgcagctgaaagccttgaagccgggagttattcaaatcttgggagtcaagacatccaggttcctgtgccagcggccagatggggccctgtatggatcgctccactttgaccctgaggcctgcagcttccgggagctgcttcttgaggacggatacaatgtttaccagtccgaagcccacggcctcccgctgcacctgccagggaacaagtccccacaccgggaccctgcaccccgaggaccagctcgcttcctgccactaccaggcctgccacccgcacccccggagccacccggaatcctggccccccagccccccgatgtgggctcctcggaccctctgagcatggtgggaccttcccagggccgaagccccagctacgcttccggtggaggtggtggttctggtggtggtagcggtggtggtggatccgacaaaactcacacatgcccaccgtgcccagcacctgaactcctggggggaccgtcagtcttcctcttccccccaaaacccaaggacaccctcatgatctcccgtacccctgaggtcacatgcgtggtggtggacgtgagccacgaagaccctgaggtcaagttcaactggtacgtggacggcgtggaggtgcataatgccaagacaaagccgcgtgaggagcagtacaacagcacgtaccgtgtggtcagcgtcctcaccgtcctgcaccaggactggctgaatggcaaggagtacaagtgcaaggtctccaacaaagccctcccagcccccatcgagaaaaccatctccaaagccaaagggcagccccgagaaccacaggtgtacaccctgcccccatcccgggatgagctgaccaagaaccaggtcagcctgacctgcctggtcaaaggcttctatcccagcgacatcgccgtggagtgggagagcaatgggcagccggagaacaactacaagaccacgcctcccgtgctggactccgacggctccttcttcctctatagcaagctcaccgtggacaagagcaggtggcagcaggggaacgtcttctcatgctccgtgatgcatgaggctctgcacaaccactacacgcagaagagcctctccctgtctccgggtaaa

SEQ ID NO: 41 - protein, 424 aa, Artificial Sequence
  Synthetic Construct
MHPIPDSSPLLQFGGQVRQRYLYTDDAQQTEAHLEIREDGTVGGAADQSPESLLQLKALKPGVIQILGVKTSRFLCQRPDGALYGSLHFDPEACSFRELLLEDGYNVYQSEAHGLPLHLPGNKSPHRDPAPRGPARFLPLPGLPPAPPEPPGILAPQPPDVGSSDPLSMVGPSQGRSPSYASGGGGGSGGGSGGGGSDKTHTCPPCPAPELLGGPSVFLFPPKPKDTLMISRTPEVTCVVVDVSHEDPEVKFNWYVDGVEVHNAKTKPREEQYNSTYRVVSVLTVLHQDWLNGKEYKCKVSNKALPAPIEKTISKAKGQPREPQVYTLPPSRDELTKNQVSLTCLVKGFYPSDIAVEWESNGQPENNYKTTPPVLDSDGSFFLYSKLTVDKSRWQQGNVFSCSVMHEALHNHYTQKSLSLSPGK

SEQ ID NO: 42 - DNA, 1275 bp, Artificial
  Fc L15 RG
  CDS (1)..(1275)
atggacaaaactcacacatgtccaccttgtccagctccggaactcctggggggaccgtcagtcttcctcttccccccaaaacccaaggacaccctcatgatctcccgtacccctgaggtcacatgcgtggtggtggacgtgagccacgaagaccctgaggtcaagttcaactggtacgtggacggcgtggaggtgcataatgccaagacaaagccgcgtgaggagcagtacaacagcacgtaccgtgtggtcagcgtcctcaccgtcctgcaccaggactggctgaatggcaaggagtacaagtgcaaggtctccaacaaagccctcccagcccccatcgagaaaaccatctccaaagccaaagggcagccccgagaaccacaggtgtacaccctgcccccatcccgtgatgagctgaccaagaaccaggtcagcctgacctgcctggtcaaaggcttctatcccagcgacatcgccgtggagtgggagagcaatgggcagccggagaacaactacaagaccacgcctcccgtgctggactccgacggctccttcttcctctacagcaagctcaccgtggacaagagccgttggcagcaggggaacgtcttctcatgctccgtgatgcatgaggctctgcacaaccactacacgcagaagagcctctccctgtctccgggtaaaggtggaggtggtggttctggtggtggtagcggtggtggtggatcccatccaattccagattcttctccattattacaattcgggggccaagtccggcagcggtacctctacacagatgatgcccagcagacagaagcccacctggagatcagggaggatgggacggtggggggcgctgctgaccagagccccgaaagtctcctgcagctgaaagccttgaagccgggagttattcaaatcttgggagtcaagacatccaggttcctgtgccagcggccagatggggccctgtatggatcgctccactttgaccctgaggcctgcagcttccgggagcgtcttcttgaggacggatacaatgtttaccagtccgaagcccacggcctcccgctgcacctgccagggaacaagtccccacaccgggaccctgcaccccgaggaccagctcgcttcctgccactaccaggcctgccccccgcacccccggagccacccggaatcctggccccccagccccccgatgtgggctcctcggaccctctgagcatggtgggaggttcccagggccgaagccccagctacgcttcctaa

SEQ ID NO: 43 - protein, 424 aa, Artificial
  Synthetic Construct
MDKTHTCPPCPAPELLGGPSVFLFPPKPKDTLMISRTPEVTCVVVDVSHEDPEVKFNWYVDGVEVHNAKTKPREEQYNSTYRVVSVLTVLHQDWLNGKEYKCKVSNKALPAPIEKTISKAKGQPREPQVYTLPPSRDELTKNQVSLTCLVKGFYPSDIAVEWESNGQPENNYKTTPPVLDSDGSFFLYSKLTVDKSRWQQGNVFSCSVMHEALHNHYTQKSLSLSPGKGGGGGSGGGSGGGGSHPIPDSSPLLQFGGQVRQRYLYTDDAQQTEAHLEIREDGTVGGAADQSPESLLQLKALKPGVIQILGVKTSRFLCQRPDGALYGSLHFDPEACSFRERLLEDGYNVYQSEAHGLPLHLPGNKSPHRDPAPRGPARFLPLPGLPPAPPEPPGILAPQPPDVGSSDPLSMVGGSQGRSPSYAS

SEQ ID NO: 44 - DNA, 1275 bp, Artificial Sequence
  Fc-(G4S)3-RG
  CDS (1)..(1275)
atggacaaaactcacacatgtccaccttgtccagctccggaactcctggggggaccgtcagtcttcctcttccccccaaaacccaaggacaccctcatgatctcccgtacccctgaggtcacatgcgtggtggtggacgtgagccacgaagaccctgaggtcaagttcaactggtacgtggacggcgtggaggtgcataatgccaagacaaagccgcgtgaggagcagtacaacagcacgtaccgtgtggtcagcgtcctcaccgtcctgcaccaggactggctgaatggcaaggagtacaagtgcaaggtctccaacaaagccctcccagcccccatcgagaaaaccatctccaaagccaaagggcagccccgagaaccacaggtgtacaccctgcccccatcccgtgatgagctgaccaagaaccaggtcagcctgacctgcctggtcaaaggcttctatcccagcgacatcgccgtggagtgggagagcaatgggcagccggagaacaactacaagaccacgcctcccgtgctggactccgacggctccttcttcctctacagcaagctcaccgtggacaagagccgttggcagcaggggaacgtcttctcatgctccgtgatgcatgaggctctgcacaaccactacacgcagaagagcctctccctgtctccgggtaaaggtggtggtggttccggtggcggcggctctggtggtggtggcagccatccgatcccggactcttctccgctgctgcagttcggtggtcaggttcgtcagcgttacctgtacaccgacgacgcgcagcagaccgaggcgcacctggagatccgtgaagacggtaccgttggtggtgcggccgaccagtctccggaatctctgctgcagctgaaagccctgaaaccgggtgttatccagatcctgggcgttaaaacctctcgtttcctgtgccagcgtccggacggcgccctgtacggttctctgcacttcgacccggaggcgtgctcttttcgtgaacgtctgctcgaagacggttacaacgtttaccagtctgaggcgcacggtctgccgctgcacctgccgggtaacaaatctccgcaccgtgacccggcgccacgtggtcctgcgcgtttcctgccactgccgggcctgccgcctgcgcctcctgaaccgcctggtatcctggctccgcagccgccagacgttggttcttctgacccgctgtctatggttggtggctctcagggtcgttctccgtcttacgcctcttaa

SEQ ID NO: 45 - protein, 424 aa, Artificial Sequence
  Synthetic Construct
MDKTHTCPPCPAPELLGGPSVFLFPPKPKDTLMISRTPEVTCVVVDVSHEDPEVKFNWYVDGVEVHNAKTKPREEQYNSTYRVVSVLTVLHQDWLNGKEYKCKVSNKALPAPIEKTISKAKGQPREPQVYTLPPSRDELTKNQVSLTCLVKGFYPSDIAVEWESNGQPENNYKTTPPVLDSDGSFFLYSKLTVDKSRWQQGNVFSCSVMHEALHNHYTQKSLSLSPGKGGGGSGGGGSGGGGSHPIPDSSPLLQFGGQVRQRYLYTDDAQQTEAHLEIREDGTVGGAADQSPESLLQLKALKPGVIQILGVKTSRFLCQRPDGALYGSLHFDPEACSFRERLLEDGYNVYQSEAHGLPLHLPGNKSPHRDPAPRGPARFLPLPGLPPAPPEPPGILAPQPPDVGSSDPLSMVGGSQGRSPSYAS

SEQ ID NO: 46 - DNA, 1275 bp, Artificial
  Fc-(G4S)3-RGE
  CDS (1)..(1275)
atggacaaaactcacacatgtccaccttgtccagctccggaactcctggggggaccgtcagtcttcctcttccccccaaaacccaaggacaccctcatgatctcccgtacccctgaggtcacatgcgtggtggtggacgtgagccacgaagaccctgaggtcaagttcaactggtacgtggacggcgtggaggtgcataatgccaagacaaagccgcgtgaggagcagtacaacagcacgtaccgtgtggtcagcgtcctcaccgtcctgcaccaggactggctgaatggcaaggagtacaagtgcaaggtctccaacaaagccctcccagcccccatcgagaaaaccatctccaaagccaaagggcagccccgagaaccacaggtgtacaccctgcccccatcccgtgatgagctgaccaagaaccaggtcagcctgacctgcctggtcaaaggcttctatcccagcgacatcgccgtggagtgggagagcaatgggcagccggagaacaactacaagaccacgcctcccgtgctggactccgacggctccttcttcctctacagcaagctcaccgtggacaagagccgttggcagcaggggaacgtcttctcatgctccgtgatgcatgaggctctgcacaaccactacacgcagaagagcctctccctgtctccgggtaaaggtggtggtggttctggtggtggtggtagcggtggtggtggttcccatccaattccagattcttctccattattacaattcgggggccaagtccggcagcgttacctctacacagatgatgcccagcagacagaagcccacctggagatcagggaggacgggacggtggggggtgctgctgaccagagccccgaaagtctcctgcagctgaaagccttgaagccgggtgttattcaaatcttgggtgtcaagacatccaggttcctgtgccagcggccagatggggccctgtatggatcgctccactttgaccctgaggcctgcagcttccgtgagcgtcttcttgaggacggttacaatgtttaccagtccgaagcccacggcctcccgctgcacctgccagggaacaagtccccacaccgtgaccctgcaccccgaggaccagctcgcttcctgccactaccaggcctgccccccgcacccccggagccacccggaatcctggccccccagccccccgatgtgggctcctcggaccctctgagcatggtgggtggttcccagggccgaagccccagctacgaatcctaa

SEQ ID NO: 47 - protein, 424 aa, Artificial
  Synthetic Construct
MDKTHTCPPCPAPELLGGPSVFLFPPKPKDTLMISRTPEVTCVVVDVSHEDPEVKFNWYVDGVEVHNAKTKPREEQYNSTYRVVSVLTVLHQDWLNGKEYKCKVSNKALPAPIEKTISKAKGQPREPQVYTLPPSRDELTKNQVSLTCLVKGFYPSDIAVEWESNGQPENNYKTTPPVLDSDGSFFLYSKLTVDKSRWQQGNVFSCSVMHEALHNHYTQKSLSLSPGKGGGGSGGGGSGGGGSHPIPDSSPLLQFGGQVRQRYLYTDDAQQTEAHLEIREDGTVGGAADQSPESLLQLKALKPGVIQILGVKTSRFLCQRPDGALYGSLHFDPEACSFRERLLEDGYNVYQSEAHGLPLHLPGNKSPHRDPAPRGPARFLPLPGLPPAPPEPPGILAPQPPDVGSSDPLSMVGGSQGRSPSYES

SEQ ID NO: 48 - DNA, 1275 bp, Artificial Sequence
  Fc-L15-WT21
  CDS (1)..(1275)
atggacaaaactcacacatgtccaccttgtccagctccggaactcctggggggaccgtcagtcttcctcttccccccaaaacccaaggacaccctcatgatctcccgtacccctgaggtcacatgcgtggtggtggacgtgagccacgaagaccctgaggtcaagttcaactggtacgtggacggcgtggaggtgcataatgccaagacaaagccgcgtgaggagcagtacaacagcacgtaccgtgtggtcagcgtcctcaccgtcctgcaccaggactggctgaatggcaaggagtacaagtgcaaggtctccaacaaagccctcccagcccccatcgagaaaaccatctccaaagccaaagggcagccccgagaaccacaggtgtacaccctgcccccatcccgtgatgagctgaccaagaaccaggtcagcctgacctgcctggtcaaaggcttctatcccagcgacatcgccgtggagtgggagagcaatgggcagccggagaacaactacaagaccacgcctcccgtgctggactccgacggctccttcttcctctacagcaagctcaccgtggacaagagccgttggcagcaggggaacgtcttctcatgctccgtgatgcatgaggctctgcacaaccactacacgcagaagagcctctccctgtctccgggtaaaggtggaggtggtggttctggtggtggtagcggtggtggtggatcccatccaattccagattcttctccattattacaattcgggggccaagtccggcagcggtacctctacacagatgatgcccagcagacagaagcccacctggagatcagggaggatgggacggtggggggcgctgctgaccagagccccgaaagtctcctgcagctgaaagccttgaagccgggagttattcaaatcttgggagtcaagacatccaggttcctgtgccagcggccagatggggccctgtatggatcgctccactttgaccctgaggcctgcagcttccgggagctgcttcttgaggacggatacaatgtttaccagtccgaagcccacggcctcccgctgcacctgccagggaacaagtccccacaccgggaccctgcaccccgaggaccagctcgcttcctgccactaccaggcctgccccccgcacccccggagccacccggaatcctggccccccagccccccgatgtgggctcctcggaccctctgagcatggtgggaccttcccagggccgaagccccagctacgcttcctaa

SEQ ID NO: 49 - protein, 424 aa, Artificial Sequence
  Synthetic Construct
MDKTHTCPPCPAPELLGGPSVFLFPPKPKDTLMISRTPEVTCVVVDVSHEDPEVKFNWYVDGVEVHNAKTKPREEQYNSTYRVVSVLTVLHQDWLNGKEYKCKVSNKALPAPIEKTISKAKGQPREPQVYTLPPSRDELTKNQVSLTCLVKGFYPSDIAVEWESNGQPENNYKTTPPVLDSDGSFFLYSKLTVDKSRWQQGNVFSCSVMHEALHNHYTQKSLSLSPGKGGGGGSGGGSGGGGSHPIPDSSPLLQFGGQVRQRYLYTDDAQQTEAHLEIREDGTVGGAADQSPESLLQLKALKPGVIQILGVKTSRFLCQRPDGALYGSLHFDPEACSFRELLLEDGYNVYQSEAHGLPLHLPGNKSPHRDPAPRGPARFLPLPGLPPAPPEPPGILAPQPPDVGSSDPLSMVGPSQGRSPSYAS

SEQ ID NO: 50 - DNA, 1275 bp, Artificial Sequence
  Fc-L15-G170E
  CDS (1)..(1275)
atggacaaaactcacacatgtccaccttgtccagctccggaactcctggggggaccgtcagtcttcctcttccccccaaaacccaaggacaccctcatgatctcccgtacccctgaggtcacatgcgtggtggtggacgtgagccacgaagaccctgaggtcaagttcaactggtacgtggacggcgtggaggtgcataatgccaagacaaagccgcgtgaggagcagtacaacagcacgtaccgtgtggtcagcgtcctcaccgtcctgcaccaggactggctgaatggcaaggagtacaagtgcaaggtctccaacaaagccctcccagcccccatcgagaaaaccatctccaaagccaaagggcagccccgagaaccacaggtgtacaccctgcccccatcccgtgatgagctgaccaagaaccaggtcagcctgacctgcctggtcaaaggcttctatcccagcgacatcgccgtggagtgggagagcaatgggcagccggagaacaactacaagaccacgcctcccgtgctggactccgacggctccttcttcctctacagcaagctcaccgtggacaagagccgttggcagcaggggaacgtcttctcatgctccgtgatgcatgaggctctgcacaaccactacacgcagaagagcctctccctgtctccgggtaaaggtggaggtggtggttctggtggtggtagcggtggtggtggatcccatccaattccagattcttctccattattacaattcgggggccaagtccggcagcggtacctctacacagatgatgcccagcagacagaagcccacctggagatcagggaggatgggacggtggggggcgctgctgaccagagccccgaaagtctcctgcagctgaaagccttgaagccgggagttattcaaatcttgggagtcaagacatccaggttcctgtgccagcggccagatggggccctgtatggatcgctccactttgaccctgaggcctgcagcttccgggagctgcttcttgaggacggatacaatgtttaccagtccgaagcccacggcctcccgctgcacctgccagggaacaagtccccacaccgggaccctgcaccccgaggaccagctcgcttcctgccactaccaggcctgccccccgcacccccggagccacccggaatcctggccccccagccccccgatgtgggctcctcggaccctctgagcatggtggaaccttcccagggccgaagccccagctacgcttcctaa

SEQ ID NO: 51 - protein, 424 aa, Artificial Sequence
  Synthetic Construct
MDKTHTCPPCPAPELLGGPSVFLFPPKPKDTLMISRTPEVTCVVVDVSHEDPEVKFNWYVDGVEVHNAKTKPREEQYNSTYRVVSVLTVLHQDWLNGKEYKCKVSNKALPAPIEKTISKAKGQPREPQVYTLPPSRDELTKNQVSLTCLVKGFYPSDIAVEWESNGQPENNYKTTPPVLDSDGSFFLYSKLTVDKSRWQQGNVFSCSVMHEALHNHYTQKSLSLSPGKGGGGGSGGGSGGGGSHPIPDSSPLLQFGGQVRQRYLYTDDAQQTEAHLEIREDGTVGGAADQSPESLLQLKALKPGVIQILGVKTSRFLCQRPDGALYGSLHFDPEACSFRELLLEDGYNVYQSEAHGLPLHLPGNKSPHRDPAPRGPARFLPLPGLPPAPPEPPGILAPQPPDVGSSDPLSMVEPSQGRSPSYAS

SEQ ID NO: 52 - DNA, 1275 bp, Artificial Sequence
  Fc-L15-P171A
  CDS (1)..(1275)
atggacaaaactcacacatgtccaccttgtccagctccggaactcctggggggaccgtcagtcttcctcttccccccaaaacccaaggacaccctcatgatctcccgtacccctgaggtcacatgcgtggtggtggacgtgagccacgaagaccctgaggtcaagttcaactggtacgtggacggcgtggaggtgcataatgccaagacaaagccgcgtgaggagcagtacaacagcacgtaccgtgtggtcagcgtcctcaccgtcctgcaccaggactggctgaatggcaaggagtacaagtgcaaggtctccaacaaagccctcccagcccccatcgagaaaaccatctccaaagccaaagggcagccccgagaaccacaggtgtacaccctgcccccatcccgtgatgagctgaccaagaaccaggtcagcctgacctgcctggtcaaaggcttctatcccagcgacatcgccgtggagtgggagagcaatgggcagccggagaacaactacaagaccacgcctcccgtgctggactccgacggctccttcttcctctacagcaagctcaccgtggacaagagccgttggcagcaggggaacgtcttctcatgctccgtgatgcatgaggctctgcacaaccactacacgcagaagagcctctccctgtctccgggtaaaggtggaggtggtggttctggtggtggtagcggtggtggtggatcccatccaattccagattcttctccattattacaattcgggggccaagtccggcagcggtacctctacacagatgatgcccagcagacagaagcccacctggagatcagggaggatgggacggtggggggcgctgctgaccagagccccgaaagtctcctgcagctgaaagccttgaagccgggagttattcaaatcttgggagtcaagacatccaggttcctgtgccagcggccagatggggccctgtatggatcgctccactttgaccctgaggcctgcagcttccgggagctgcttcttgaggacggatacaatgtttaccagtccgaagcccacggcctcccgctgcacctgccagggaacaagtccccacaccgggaccctgcaccccgaggaccagctcgcttcctgccactaccaggcctgccccccgcacccccggagccacccggaatcctggccccccagccccccgatgtgggctcctcggaccctctgagcatggtgggagcttcccagggccgaagccccagctacgcttcctaa

SEQ ID NO: 53 - protein, 424 aa, Artificial Sequence
  Synthetic Construct
MDKTHTCPPCPAPELLGGPSVFLFPPKPKDTLMISRTPEVTCVVVDVSHEDPEVKFNWYVDGVEVHNAKTKPREEQYNSTYRVVSVLTVLHQDWLNGKEYKCKVSNKALPAPIEKTISKAKGQPREPQVYTLPPSRDELTKNQVSLTCLVKGFYPSDIAVEWESNGQPENNYKTTPPVLDSDGSFFLYSKLTVDKSRWQQGNVFSCSVMHEALHNHYTQKSLSLSPGKGGGGGSGGGSGGGGSHPIPDSSPLLQFGGQVRQRYLYTDDAQQTEAHLEIREDGTVGGAADQSPESLLQLKALKPGVIQILGVKTSRFLCQRPDGALYGSLHFDPEACSFRELLLEDGYNVYQSEAHGLPLHLPGNKSPHRDPAPRGPARFLPLPGLPPAPPEPPGILAPQPPDVGSSDPLSMVGASQGRSPSYAS

SEQ ID NO: 54 - DNA, 1275 bp, Artificial Sequence
  Fc-L15-S172L
  CDS (1)..(1275)
atggacaaaactcacacatgtccaccttgtccagctccggaactcctggggggaccgtcagtcttcctcttccccccaaaacccaaggacaccctcatgatctcccgtacccctgaggtcacatgcgtggtggtggacgtgagccacgaagaccctgaggtcaagttcaactggtacgtggacggcgtggaggtgcataatgccaagacaaagccgcgtgaggagcagtacaacagcacgtaccgtgtggtcagcgtcctcaccgtcctgcaccaggactggctgaatggcaaggagtacaagtgcaaggtctccaacaaagccctcccagcccccatcgagaaaaccatctccaaagccaaagggcagccccgagaaccacaggtgtacaccctgcccccatcccgtgatgagctgaccaagaaccaggtcagcctgacctgcctggtcaaaggcttctatcccagcgacatcgccgtggagtgggagagcaatgggcagccggagaacaactacaagaccacgcctcccgtgctggactccgacggctccttcttcctctacagcaagctcaccgtggacaagagccgttggcagcaggggaacgtcttctcatgctccgtgatgcatgaggctctgcacaaccactacacgcagaagagcctctccctgtctccgggtaaaggtggaggtggtggttctggtggtggtagcggtggtggtggatcccatccaattccagattcttctccattattacaattcgggggccaagtccggcagcggtacctctacacagatgatgcccagcagacagaagcccacctggagatcagggaggatgggacggtggggggcgctgctgaccagagccccgaaagtctcctgcagctgaaagccttgaagccgggagttattcaaatcttgggagtcaagacatccaggttcctgtgccagcggccagatggggccctgtatggatcgctccactttgaccctgaggcctgcagcttccgggagctgcttcttgaggacggatacaatgtttaccagtccgaagcccacggcctcccgctgcacctgccagggaacaagtccccacaccgggaccctgcaccccgaggaccagctcgcttcctgccactaccaggcctgccccccgcacccccggagccacccggaatcctggccccccagccccccgatgtgggctcctcggaccctctgagcatggtgggacctctgcagggccgaagccccagctacgcttcctaa

SEQ ID NO: 55 - protein, 424 aa, Artificial Sequence
  Synthetic Construct
MDKTHTCPPCPAPELLGGPSVFLFPPKPKDTLMISRTPEVTCVVVDVSHEDPEVKFNWYVDGVEVHNAKTKPREEQYNSTYRVVSVLTVLHQDWLNGKEYKCKVSNKALPAPIEKTISKAKGQPREPQVYTLPPSRDELTKNQVSLTCLVKGFYPSDIAVEWESNGQPENNYKTTPPVLDSDGSFFLYSKLTVDKSRWQQGNVFSCSVMHEALHNHYTQKSLSLSPGKGGGGGSGGGSGGGGSHPIPDSSPLLQFGGQVRQRYLYTDDAQQTEAHLEIREDGTVGGAADQSPESLLQLKALKPGVIQILGVKTSRFLCQRPDGALYGSLHFDPEACSFRELLLEDGYNVYQSEAHGLPLHLPGNKSPHRDPAPRGPARFLPLPGLPPAPPEPPGILAPQPPDVGSSDPLSMVGPLQGRSPSYAS

SEQ ID NO: 56 - DNA, 1275 bp, Artificial Sequence
  Fc-L15-RGE
  CDS (1)..(1275)
atggacaaaactcacacatgtccaccttgtccagctccggaactcctggggggaccgtcagtcttcctcttccccccaaaacccaaggacaccctcatgatctcccgtacccctgaggtcacatgcgtggtggtggacgtgagccacgaagaccctgaggtcaagttcaactggtacgtggacggcgtggaggtgcataatgccaagacaaagccgcgtgaggagcagtacaacagcacgtaccgtgtggtcagcgtcctcaccgtcctgcaccaggactggctgaatggcaaggagtacaagtgcaaggtctccaacaaagccctcccagcccccatcgagaaaaccatctccaaagccaaagggcagccccgagaaccacaggtgtacaccctgcccccatcccgtgatgagctgaccaagaaccaggtcagcctgacctgcctggtcaaaggcttctatcccagcgacatcgccgtggagtgggagagcaatgggcagccggagaacaactacaagaccacgcctcccgtgctggactccgacggctccttcttcctctacagcaagctcaccgtggacaagagccgttggcagcaggggaacgtcttctcatgctccgtgatgcatgaggctctgcacaaccactacacgcagaagagcctctccctgtctccgggtaaaggtggtggtggtggttctggtggtggtagcggtggtggtggttcccatccaattccagattcttctccattattacaattcgggggccaagtccggcagcgttacctctacacagatgatgcccagcagacagaagcccacctggagatcagggaggacgggacggtggggggtgctgctgaccagagccccgaaagtctcctgcagctgaaagccttgaagccgggtgttattcaaatcttgggtgtcaagacatccaggttcctgtgccagcggccagatggggccctgtatggatcgctccactttgaccctgaggcctgcagcttccgtgagcgtcttcttgaggacggttacaatgtttaccagtccgaagcccacggcctcccgctgcacctgccagggaacaagtccccacaccgtgaccctgcaccccgaggaccagctcgcttcctgccactaccaggcctgccccccgcacccccggagccacccggaatcctggccccccagccccccgatgtgggctcctcggaccctctgagcatggtgggtggttcccagggccgaagccccagctacgaatcctaa

SEQ ID NO: 57 - protein, 424 aa, Artificial Sequence
  Synthetic Construct
MDKTHTCPPCPAPELLGGPSVFLFPPKPKDTLMISRTPEVTCVVVDVSHEDPEVKFNWYVDGVEVHNAKTKPREEQYNSTYRVVSVLTVLHQDWLNGKEYKCKVSNKALPAPIEKTISKAKGQPREPQVYTLPPSRDELTKNQVSLTCLVKGFYPSDIAVEWESNGQPENNYKTTPPVLDSDGSFFLYSKLTVDKSRWQQGNVFSCSVMHEALHNHYTQKSLSLSPGKGGGGGSGGGSGGGGSHPIPDSSPLLQFGGQVRQRYLYTDDAQQTEAHLEIREDGTVGGAADQSPESLLQLKALKPGVIQILGVKTSRFLCQRPDGALYGSLHFDPEACSFRERLLEDGYNVYQSEAHGLPLHLPGNKSPHRDPAPRGPARFLPLPGLPPAPPEPPGILAPQPPDVGSSDPLSMVGGSQGRSPSYES

SEQ ID NO: 58 - DNA, 1275 bp, Artificial Sequence
  Fc-L15-G170E P171A S172L
  CDS (1)..(1275)
atggacaaaactcacacatgtccaccttgtccagctccggaactcctggggggaccgtcagtcttcctcttccccccaaaacccaaggacaccctcatgatctcccgtacccctgaggtcacatgcgtggtggtggacgtgagccacgaagaccctgaggtcaagttcaactggtacgtggacggcgtggaggtgcataatgccaagacaaagccgcgtgaggagcagtacaacagcacgtaccgtgtggtcagcgtcctcaccgtcctgcaccaggactggctgaatggcaaggagtacaagtgcaaggtctccaacaaagccctcccagcccccatcgagaaaaccatctccaaagccaaagggcagccccgagaaccacaggtgtacaccctgcccccatcccgtgatgagctgaccaagaaccaggtcagcctgacctgcctggtcaaaggcttctatcccagcgacatcgccgtggagtgggagagcaatgggcagccggagaacaactacaagaccacgcctcccgtgctggactccgacggctccttcttcctctacagcaagctcaccgtggacaagagccgttggcagcaggggaacgtcttctcatgctccgtgatgcatgaggctctgcacaaccactacacgcagaagagcctctccctgtctccgggtaaaggtggaggtggtggttctggtggtggtagcggtggtggtggatcccatccaattccagattcttctccattattacaattcgggggccaagtccggcagcggtacctctacacagatgatgcccagcagacagaagcccacctggagatcagggaggatgggacggtggggggcgctgctgaccagagccccgaaagtctcctgcagctgaaagccttgaagccgggagttattcaaatcttgggagtcaagacatccaggttcctgtgccagcggccagatggggccctgtatggatcgctccactttgaccctgaggcctgcagcttccgggagctgcttcttgaggacggatacaatgtttaccagtccgaagcccacggcctcccgctgcacctgccagggaacaagtccccacaccgggaccctgcaccccgaggaccagctcgcttcctgccactaccaggcctgccccccgcacccccggagccacccggaatcctggccccccagccccccgatgtgggctcctcggaccctctgagcatggtggaagctctgcagggccgaagccccagctacgcttcctaa

SEQ ID NO: 59 - protein, 424 aa, Artificial Sequence
  Synthetic Construct
MDKTHTCPPCPAPELLGGPSVFLFPPKPKDTLMISRTPEVTCVVVDVSHEDPEVKFNWYVDGVEVHNAKTKPREEQYNSTYRVVSVLTVLHQDWLNGKEYKCKVSNKALPAPIEKTISKAKGQPREPQVYTLPPSRDELTKNQVSLTCLVKGFYPSDIAVEWESNGQPENNYKTTPPVLDSDGSFFLYSKLTVDKSRWQQGNVFSCSVMHEALHNHYTQKSLSLSPGKGGGGGSGGGSGGGGSHPIPDSSPLLQFGGQVRQRYLYTDDAQQTEAHLEIREDGTVGGAADQSPESLLQLKALKPGVIQILGVKTSRFLCQRPDGALYGSLHFDPEACSFRELLLEDGYNVYQSEAHGLPLHLPGNKSPHRDPAPRGPARFLPLPGLPPAPPEPPGILAPQPPDVGSSDPLSMVEALQGRSPSYAS

SEQ ID NO: 60 - DNA, 1275 bp, Artificial Sequence
  Fc-L15-G151A
  CDS (1)..(1275)
atggacaaaactcacacatgtccaccttgtccagctccggaactcctggggggaccgtcagtcttcctcttccccccaaaacccaaggacaccctcatgatctcccgtacccctgaggtcacatgcgtggtggtggacgtgagccacgaagaccctgaggtcaagttcaactggtacgtggacggcgtggaggtgcataatgccaagacaaagccgcgtgaggagcagtacaacagcacgtaccgtgtggtcagcgtcctcaccgtcctgcaccaggactggctgaatggcaaggagtacaagtgcaaggtctccaacaaagccctcccagcccccatcgagaaaaccatctccaaagccaaagggcagccccgagaaccacaggtgtacaccctgcccccatcccgtgatgagctgaccaagaaccaggtcagcctgacctgcctggtcaaaggcttctatcccagcgacatcgccgtggagtgggagagcaatgggcagccggagaacaactacaagaccacgcctcccgtgctggactccgacggctccttcttcctctacagcaagctcaccgtggacaagagccgttggcagcaggggaacgtcttctcatgctccgtgatgcatgaggctctgcacaaccactacacgcagaagagcctctccctgtctccgggtaaaggtggaggtggtggttctggtggtggtagcggtggtggtggatcccatccaattccagattcttctccattattacaattcgggggccaagtccggcagcggtacctctacacagatgatgcccagcagacagaagcccacctggagatcagggaggatgggacggtggggggcgctgctgaccagagccccgaaagtctcctgcagctgaaagccttgaagccgggagttattcaaatcttgggagtcaagacatccaggttcctgtgccagcggccagatggggccctgtatggatcgctccactttgaccctgaggcctgcagcttccgggagctgcttcttgaggacggatacaatgtttaccagtccgaagcccacggcctcccgctgcacctgccagggaacaagtccccacaccgggaccctgcaccccgaggaccagctcgcttcctgccactaccaggcctgccccccgcacccccggagccacccgcaatcctggccccccagccccccgatgtgggctcctcggaccctctgagcatggtgggaccttcccagggccgaagccccagctacgcttcctaa

SEQ ID NO: 61 - protein, 424 aa, Artificial Sequence
  Synthetic Construct
MDKTHTCPPCPAPELLGGPSVFLFPPKPKDTLMISRTPEVTCVVVDVSHEDPEVKFNWYVDGVEVHNAKTKPREEQYNSTYRVVSVLTVLHQDWLNGKEYKCKVSNKALPAPIEKTISKAKGQPREPQVYTLPPSRDELTKNQVSLTCLVKGFYPSDIAVEWESNGQPENNYKTTPPVLDSDGSFFLYSKLTVDKSRWQQGNVFSCSVMHEALHNHYTQKSLSLSPGKGGGGGSGGGSGGGGSHPIPDSSPLLQFGGQVRQRYLYTDDAQQTEAHLEIREDGTVGGAADQSPESLLQLKALKPGVIQILGVKTSRFLCQRPDGALYGSLHFDPEACSFRELLLEDGYNVYQSEAHGLPLHLPGNKSPHRDPAPRGPARFLPLPGLPPAPPEPPAILAPQPPDVGSSDPLSMVGPSQGRSPSYAS

SEQ ID NO: 62 - DNA, 1275 bp, Artificial Sequence
  Fc-L15-G170E P171A
  CDS (1)..(1275)
atggacaaaactcacacatgtccaccttgtccagctccggaactcctggggggaccgtcagtcttcctcttccccccaaaacccaaggacaccctcatgatctcccgtacccctgaggtcacatgcgtggtggtggacgtgagccacgaagaccctgaggtcaagttcaactggtacgtggacggcgtggaggtgcataatgccaagacaaagccgcgtgaggagcagtacaacagcacgtaccgtgtggtcagcgtcctcaccgtcctgcaccaggactggctgaatggcaaggagtacaagtgcaaggtctccaacaaagccctcccagcccccatcgagaaaaccatctccaaagccaaagggcagccccgagaaccacaggtgtacaccctgcccccatcccgtgatgagctgaccaagaaccaggtcagcctgacctgcctggtcaaaggcttctatcccagcgacatcgccgtggagtgggagagcaatgggcagccggagaacaactacaagaccacgcctcccgtgctggactccgacggctccttcttcctctacagcaagctcaccgtggacaagagccgttggcagcaggggaacgtcttctcatgctccgtgatgcatgaggctctgcacaaccactacacgcagaagagcctctccctgtctccgggtaaaggtggaggtggtggttctggtggtggtagcggtggtggtggatcccatccaattccagattcttctccattattacaattcgggggccaagtccggcagcggtacctctacacagatgatgcccagcagacagaagcccacctggagatcagggaggatgggacggtggggggcgctgctgaccagagccccgaaagtctcctgcagctgaaagccttgaagccgggagttattcaaatcttgggagtcaagacatccaggttcctgtgccagcggccagatggggccctgtatggatcgctccactttgaccctgaggcctgcagcttccgggagctgcttcttgaggacggatacaatgtttaccagtccgaagcccacggcctcccgctgcacctgccagggaacaagtccccacaccgggaccctgcaccccgaggaccagctcgcttcctgccactaccaggcctgccccccgcacccccggagccacccggaatcctggccccccagccccccgatgtgggctcctcggaccctctgagcatggtggaagcttcccagggccgaagccccagctacgcttcctaa

SEQ ID NO: 63 - protein, 424 aa, Artificial Sequence
  Synthetic Construct
MDKTHTCPPCPAPELLGGPSVFLFPPKPKDTLMISRTPEVTCVVVDVSHEDPEVKFNWYVDGVEVHNAKTKPREEQYNSTYRVVSVLTVLHQDWLNGKEYKCKVSNKALPAPIEKTISKAKGQPREPQVYTLPPSRDELTKNQVSLTCLVKGFYPSDIAVEWESNGQPENNYKTTPPVLDSDGSFFLYSKLTVDKSRWQQGNVFSCSVMHEALHNHYTQKSLSLSPGKGGGGGSGGGSGGGGSHPIPDSSPLLQFGGQVRQRYLYTDDAQQTEAHLEIREDGTVGGAADQSPESLLQLKALKPGVIQILGVKTSRFLCQRPDGALYGSLHFDPEACSFRELLLEDGYNVYQSEAHGLPLHLPGNKSPHRDPAPRGPARFLPLPGLPPAPPEPPGILAPQPPDVGSSDPLSMVEASQGRSPSYAS

SEQ ID NO: 64 - DNA, 1275 bp, Artificial Sequence
  Fc-L15-P150A G151A I152V
  CDS (1)..(1275)
atggacaaaactcacacatgtccaccttgtccagctccggaactcctggggggaccgtcagtcttcctcttccccccaaaacccaaggacaccctcatgatctcccgtacccctgaggtcacatgcgtggtggtggacgtgagccacgaagaccctgaggtcaagttcaactggtacgtggacggcgtggaggtgcataatgccaagacaaagccgcgtgaggagcagtacaacagcacgtaccgtgtggtcagcgtcctcaccgtcctgcaccaggactggctgaatggcaaggagtacaagtgcaaggtctccaacaaagccctcccagcccccatcgagaaaaccatctccaaagccaaagggcagccccgagaaccacaggtgtacaccctgcccccatcccgtgatgagctgaccaagaaccaggtcagcctgacctgcctggtcaaaggcttctatcccagcgacatcgccgtggagtgggagagcaatgggcagccggagaacaactacaagaccacgcctcccgtgctggactccgacggctccttcttcctctacagcaagctcaccgtggacaagagccgttggcagcaggggaacgtcttctcatgctccgtgatgcatgaggctctgcacaaccactacacgcagaagagcctctccctgtctccgggtaaaggtggaggtggtggttctggtggtggtagcggtggtggtggatcccatccaattccagattcttctccattattacaattcgggggccaagtccggcagcggtacctctacacagatgatgcccagcagacagaagcccacctggagatcagggaggatgggacggtggggggcgctgctgaccagagccccgaaagtctcctgcagctgaaagccttgaagccgggagttattcaaatcttgggagtcaagacatccaggttcctgtgccagcggccagatggggccctgtatggatcgctccactttgaccctgaggcctgcagcttccgggagctgcttcttgaggacggatacaatgtttaccagtccgaagcccacggcctcccgctgcacctgccagggaacaagtccccacaccgggaccctgcaccccgaggaccagctcgcttcctgccactaccaggcctgccccccgcacccccggagccagccgcagttctggccccccagccccccgatgtgggctcctcggaccctctgagcatggtgggaccttcccagggccgaagccccagctacgcttcctaa

SEQ ID NO: 65 - protein, 424 aa, Artificial Sequence
  Synthetic Construct
MDKTHTCPPCPAPELLGGPSVFLFPPKPKDTLMISRTPEVTCVVVDVSHEDPEVKFNWYVDGVEVHNAKTKPREEQYNSTYRVVSVLTVLHQDWLNGKEYKCKVSNKALPAPIEKTISKAKGQPREPQVYTLPPSRDELTKNQVSLTCLVKGFYPSDIAVEWESNGQPENNYKTTPPVLDSDGSFFLYSKLTVDKSRWQQGNVFSCSVMHEALHNHYTQKSLSLSPGKGGGGGSGGGSGGGGSHPIPDSSPLLQFGGQVRQRYLYTDDAQQTEAHLEIREDGTVGGAADQSPESLLQLKALKPGVIQILGVKTSRFLCQRPDGALYGSLHFDPEACSFRELLLEDGYNVYQSEAHGLPLHLPGNKSPHRDPAPRGPARFLPLPGLPPAPPEPAAVLAPQPPDVGSSDPLSMVGPSQGRSPSYAS

SEQ ID NO: 66 - DNA, 1275 bp, Artificial Sequence
  Fc-L15-G170E S172L
  CDS (1)..(1275)
atggacaaaactcacacatgtccaccttgtccagctccggaactcctggggggaccgtcagtcttcctcttccccccaaaacccaaggacaccctcatgatctcccgtacccctgaggtcacatgcgtggtggtggacgtgagccacgaagaccctgaggtcaagttcaactggtacgtggacggcgtggaggtgcataatgccaagacaaagccgcgtgaggagcagtacaacagcacgtaccgtgtggtcagcgtcctcaccgtcctgcaccaggactggctgaatggcaaggagtacaagtgcaaggtctccaacaaagccctcccagcccccatcgagaaaaccatctccaaagccaaagggcagccccgagaaccacaggtgtacaccctgcccccatcccgtgatgagctgaccaagaaccaggtcagcctgacctgcctggtcaaaggcttctatcccagcgacatcgccgtggagtgggagagcaatgggcagccggagaacaactacaagaccacgcctcccgtgctggactccgacggctccttcttcctctacagcaagctcaccgtggacaagagccgttggcagcaggggaacgtcttctcatgctccgtgatgcatgaggctctgcacaaccactacacgcagaagagcctctccctgtctccgggtaaaggtggaggtggtggttctggtggtggtagcggtggtggtggatcccatccaattccagattcttctccattattacaattcgggggccaagtccggcagcggtacctctacacagatgatgcccagcagacagaagcccacctggagatcagggaggatgggacggtggggggcgctgctgaccagagccccgaaagtctcctgcagctgaaagccttgaagccgggagttattcaaatcttgggagtcaagacatccaggttcctgtgccagcggccagatggggccctgtatggatcgctccactttgaccctgaggcctgcagcttccgggagctgcttcttgaggacggatacaatgtttaccagtccgaagcccacggcctcccgctgcacctgccagggaacaagtccccacaccgggaccctgcaccccgaggaccagctcgcttcctgccactaccaggcctgccccccgcacccccggagccacccggaatcctggccccccagccccccgatgtgggctcctcggaccctctgagcatggtggaacctctgcagggccgaagccccagctacgcttcctaa

SEQ ID NO: 67 - protein, 424 aa, Artificial Sequence
  Synthetic Construct
MDKTHTCPPCPAPELLGGPSVFLFPPKPKDTLMISRTPEVTCVVVDVSHEDPEVKFNWYVDGVEVHNAKTKPREEQYNSTYRVVSVLTVLHQDWLNGKEYKCKVSNKALPAPIEKTISKAKGQPREPQVYTLPPSRDELTKNQVSLTCLVKGFYPSDIAVEWESNGQPENNYKTTPPVLDSDGSFFLYSKLTVDKSRWQQGNVFSCSVMHEALHNHYTQKSLSLSPGKGGGGGSGGGSGGGGSHPIPDSSPLLQFGGQVRQRYLYTDDAQQTEAHLEIREDGTVGGAADQSPESLLQLKALKPGVIQILGVKTSRFLCQRPDGALYGSLHFDPEACSFRELLLEDGYNVYQSEAHGLPLHLPGNKSPHRDPAPRGPARFLPLPGLPPAPPEPPGILAPQPPDVGSSDPLSMVEPLQGRSPSYAS

SEQ ID NO: 68 - DNA, 1275 bp, Artificial Sequence
  Fc-L15-G170A
  CDS (1)..(1275)
atggacaaaactcacacatgtccaccttgtccagctccggaactcctggggggaccgtcagtcttcctcttccccccaaaacccaaggacaccctcatgatctcccgtacccctgaggtcacatgcgtggtggtggacgtgagccacgaagaccctgaggtcaagttcaactggtacgtggacggcgtggaggtgcataatgccaagacaaagccgcgtgaggagcagtacaacagcacgtaccgtgtggtcagcgtcctcaccgtcctgcaccaggactggctgaatggcaaggagtacaagtgcaaggtctccaacaaagccctcccagcccccatcgagaaaaccatctccaaagccaaagggcagccccgagaaccacaggtgtacaccctgcccccatcccgtgatgagctgaccaagaaccaggtcagcctgacctgcctggtcaaaggcttctatcccagcgacatcgccgtggagtgggagagcaatgggcagccggagaacaactacaagaccacgcctcccgtgctggactccgacggctccttcttcctctacagcaagctcaccgtggacaagagccgttggcagcaggggaacgtcttctcatgctccgtgatgcatgaggctctgcacaaccactacacgcagaagagcctctccctgtctccgggtaaaggtggaggtggtggttctggtggtggtagcggtggtggtggatcccatccaattccagattcttctccattattacaattcgggggccaagtccggcagcggtacctctacacagatgatgcccagcagacagaagcccacctggagatcagggaggatgggacggtggggggcgctgctgaccagagccccgaaagtctcctgcagctgaaagccttgaagccgggagttattcaaatcttgggagtcaagacatccaggttcctgtgccagcggccagatggggccctgtatggatcgctccactttgaccctgaggcctgcagcttccgggagctgcttcttgaggacggatacaatgtttaccagtccgaagcccacggcctcccgctgcacctgccagggaacaagtccccacaccgggaccctgcaccccgaggaccagctcgcttcctgccactaccaggcctgccccccgcacccccggagccacccggaatcctggccccccagccccccgatgtgggctcctcggaccctctgagcatggtggctccttcccagggccgaagccccagctacgcttcctaa

SEQ ID NO: 69 - protein, 424 aa, Artificial Sequence
  Synthetic Construct
MDKTHTCPPCPAPELLGGPSVFLFPPKPKDTLMISRTPEVTCVVVDVSHEDPEVKFNWYVDGVEVHNAKTKPREEQYNSTYRVVSVLTVLHQDWLNGKEYKCKVSNKALPAPIEKTISKAKGQPREPQVYTLPPSRDELTKNQVSLTCLVKGFYPSDIAVEWESNGQPENNYKTTPPVLDSDGSFFLYSKLTVDKSRWQQGNVFSCSVMHEALHNHYTQKSLSLSPGKGGGGGSGGGSGGGGSHPIPDSSPLLQFGGQVRQRYLYTDDAQQTEAHLEIREDGTVGGAADQSPESLLQLKALKPGVIQILGVKTSRFLCQRPDGALYGSLHFDPEACSFRELLLEDGYNVYQSEAHGLPLHLPGNKSPHRDPAPRGPARFLPLPGLPPAPPEPPGILAPQPPDVGSSDPLSMVAPSQGRSPSYAS

SEQ ID NO: 70 - DNA, 1275 bp, Artificial Sequence
  Fc-L15-G170C
  CDS (1)..(1275)
atggacaaaactcacacatgtccaccttgtccagctccggaactcctggggggaccgtcagtcttcctcttccccccaaaacccaaggacaccctcatgatctcccgtacccctgaggtcacatgcgtggtggtggacgtgagccacgaagaccctgaggtcaagttcaactggtacgtggacggcgtggaggtgcataatgccaagacaaagccgcgtgaggagcagtacaacagcacgtaccgtgtggtcagcgtcctcaccgtcctgcaccaggactggctgaatggcaaggagtacaagtgcaaggtctccaacaaagccctcccagcccccatcgagaaaaccatctccaaagccaaagggcagccccgagaaccacaggtgtacaccctgcccccatcccgtgatgagctgaccaagaaccaggtcagcctgacctgcctggtcaaaggcttctatcccagcgacatcgccgtggagtgggagagcaatgggcagccggagaacaactacaagaccacgcctcccgtgctggactccgacggctccttcttcctctacagcaagctcaccgtggacaagagccgttggcagcaggggaacgtcttctcatgctccgtgatgcatgaggctctgcacaaccactacacgcagaagagcctctccctgtctccgggtaaaggtggaggtggtggttctggtggtggtagcggtggtggtggatcccatccaattccagattcttctccattattacaattcgggggccaagtccggcagcggtacctctacacagatgatgcccagcagacagaagcccacctggagatcagggaggatgggacggtggggggcgctgctgaccagagccccgaaagtctcctgcagctgaaagccttgaagccgggagttattcaaatcttgggagtcaagacatccaggttcctgtgccagcggccagatggggccctgtatggatcgctccactttgaccctgaggcctgcagcttccgggagctgcttcttgaggacggatacaatgtttaccagtccgaagcccacggcctcccgctgcacctgccagggaacaagtccccacaccgggaccctgcaccccgaggaccagctcgcttcctgccactaccaggcctgccccccgcacccccggagccacccggaatcctggccccccagccccccgatgtgggctcctcggaccctctgagcatggtgtgcccttcccagggccgaagccccagctacgcttcctaa

SEQ ID NO: 71 - protein, 424 aa, Artificial Sequence
  Synthetic Construct
MDKTHTCPPCPAPELLGGPSVFLFPPKPKDTLMISRTPEVTCVVVDVSHEDPEVKFNWYVDGVEVHNAKTKPREEQYNSTYRVVSVLTVLHQDWLNGKEYKCKVSNKALPAPIEKTISKAKGQPREPQVYTLPPSRDELTKNQVSLTCLVKGFYPSDIAVEWESNGQPENNYKTTPPVLDSDGSFFLYSKLTVDKSRWQQGNVFSCSVMHEALHNHYTQKSLSLSPGKGGGGGSGGGSGGGGSHPIPDSSPLLQFGGQVRQRYLYTDDAQQTEAHLEIREDGTVGGAADQSPESLLQLKALKPGVIQILGVKTSRFLCQRPDGALYGSLHFDPEACSFRELLLEDGYNVYQSEAHGLPLHLPGNKSPHRDPAPRGPARFLPLPGLPPAPPEPPGILAPQPPDVGSSDPLSMVCPSQGRSPSYAS

SEQ ID NO: 72 - DNA, 1275 bp, Artificial Sequence
  Fc-L15-G170D
  CDS (1)..(1275)
atggacaaaactcacacatgtccaccttgtccagctccggaactcctggggggaccgtcagtcttcctcttccccccaaaacccaaggacaccctcatgatctcccgtacccctgaggtcacatgcgtggtggtggacgtgagccacgaagaccctgaggtcaagttcaactggtacgtggacggcgtggaggtgcataatgccaagacaaagccgcgtgaggagcagtacaacagcacgtaccgtgtggtcagcgtcctcaccgtcctgcaccaggactggctgaatggcaaggagtacaagtgcaaggtctccaacaaagccctcccagcccccatcgagaaaaccatctccaaagccaaagggcagccccgagaaccacaggtgtacaccctgcccccatcccgtgatgagctgaccaagaaccaggtcagcctgacctgcctggtcaaaggcttctatcccagcgacatcgccgtggagtgggagagcaatgggcagccggagaacaactacaagaccacgcctcccgtgctggactccgacggctccttcttcctctacagcaagctcaccgtggacaagagccgttggcagcaggggaacgtcttctcatgctccgtgatgcatgaggctctgcacaaccactacacgcagaagagcctctccctgtctccgggtaaaggtggaggtggtggttctggtggtggtagcggtggtggtggatcccatccaattccagattcttctccattattacaattcgggggccaagtccggcagcggtacctctacacagatgatgcccagcagacagaagcccacctggagatcagggaggatgggacggtggggggcgctgctgaccagagccccgaaagtctcctgcagctgaaagccttgaagccgggagttattcaaatcttgggagtcaagacatccaggttcctgtgccagcggccagatggggccctgtatggatcgctccactttgaccctgaggcctgcagcttccgggagctgcttcttgaggacggatacaatgtttaccagtccgaagcccacggcctcccgctgcacctgccagggaacaagtccccacaccgggaccctgcaccccgaggaccagctcgcttcctgccactaccaggcctgccccccgcacccccggagccacccggaatcctggccccccagccccccgatgtgggctcctcggaccctctgagcatggtggacccttcccagggccgaagccccagctacgcttcctaa

SEQ ID NO: 73 - protein, 424 aa, Artificial Sequence
  Synthetic Construct
MDKTHTCPPCPAPELLGGPSVFLFPPKPKDTLMISRTPEVTCVVVDVSHEDPEVKFNWYVDGVEVHNAKTKPREEQYNSTYRVVSVLTVLHQDWLNGKEYKCKVSNKALPAPIEKTISKAKGQPREPQVYTLPPSRDELTKNQVSLTCLVKGFYPSDIAVEWESNGQPENNYKTTPPVLDSDGSFFLYSKLTVDKSRWQQGNVFSCSVMHEALHNHYTQKSLSLSPGKGGGGGSGGGSGGGGSHPIPDSSPLLQFGGQVRQRYLYTDDAQQTEAHLEIREDGTVGGAADQSPESLLQLKALKPGVIQILGVKTSRFLCQRPDGALYGSLHFDPEACSFRELLLEDGYNVYQSEAHGLPLHLPGNKSPHRDPAPRGPARFLPLPGLPPAPPEPPGILAPQPPDVGSSDPLSMVDPSQGRSPSYAS

SEQ ID NO: 74 - DNA, 1275 bp, Artificial Sequence
  Fc-L15-G170N
  CDS (1)..(1275)
atggacaaaactcacacatgtccaccttgtccagctccggaactcctggggggaccgtcagtcttcctcttccccccaaaacccaaggacaccctcatgatctcccgtacccctgaggtcacatgcgtggtggtggacgtgagccacgaagaccctgaggtcaagttcaactggtacgtggacggcgtggaggtgcataatgccaagacaaagccgcgtgaggagcagtacaacagcacgtaccgtgtggtcagcgtcctcaccgtcctgcaccaggactggctgaatggcaaggagtacaagtgcaaggtctccaacaaagccctcccagcccccatcgagaaaaccatctccaaagccaaagggcagccccgagaaccacaggtgtacaccctgcccccatcccgtgatgagctgaccaagaaccaggtcagcctgacctgcctggtcaaaggcttctatcccagcgacatcgccgtggagtgggagagcaatgggcagccggagaacaactacaagaccacgcctcccgtgctggactccgacggctccttcttcctctacagcaagctcaccgtggacaagagccgttggcagcaggggaacgtcttctcatgctccgtgatgcatgaggctctgcacaaccactacacgcagaagagcctctccctgtctccgggtaaaggtggaggtggtggttctggtggtggtagcggtggtggtggatcccatccaattccagattcttctccattattacaattcgggggccaagtccggcagcggtacctctacacagatgatgcccagcagacagaagcccacctggagatcagggaggatgggacggtggggggcgctgctgaccagagccccgaaagtctcctgcagctgaaagccttgaagccgggagttattcaaatcttgggagtcaagacatccaggttcctgtgccagcggccagatggggccctgtatggatcgctccactttgaccctgaggcctgcagcttccgggagctgcttcttgaggacggatacaatgtttaccagtccgaagcccacggcctcccgctgcacctgccagggaacaagtccccacaccgggaccctgcaccccgaggaccagctcgcttcctgccactaccaggcctgccccccgcacccccggagccacccggaatcctggccccccagccccccgatgtgggctcctcggaccctctgagcatggtgaacccttcccagggccgaagccccagctacgcttcctaa

SEQ ID NO: 75 - protein, 424 aa, Artificial Sequence
  Synthetic Construct
MDKTHTCPPCPAPELLGGPSVFLFPPKPKDTLMISRTPEVTCVVVDVSHEDPEVKFNWYVDGVEVHNAKTKPREEQYNSTYRVVSVLTVLHQDWLNGKEYKCKVSNKALPAPIEKTISKAKGQPREPQVYTLPPSRDELTKNQVSLTCLVKGFYPSDIAVEWESNGQPENNYKTTPPVLDSDGSFFLYSKLTVDKSRWQQGNVFSCSVMHEALHNHYTQKSLSLSPGKGGGGGSGGGSGGGGSHPIPDSSPLLQFGGQVRQRYLYTDDAQQTEAHLEIREDGTVGGAADQSPESLLQLKALKPGVIQILGVKTSRFLCQRPDGALYGSLHFDPEACSFRELLLEDGYNVYQSEAHGLPLHLPGNKSPHRDPAPRGPARFLPLPGLPPAPPEPPGILAPQPPDVGSSDPLSMVNPSQGRSPSYAS

SEQ ID NO: 76 - DNA, 1275 bp, Artificial Sequence
  Fc-L15-G170S
  CDS (1)..(1275)
atggacaaaactcacacatgtccaccttgtccagctccggaactcctggggggaccgtcagtcttcctcttccccccaaaacccaaggacaccctcatgatctcccgtacccctgaggtcacatgcgtggtggtggacgtgagccacgaagaccctgaggtcaagttcaactggtacgtggacggcgtggaggtgcataatgccaagacaaagccgcgtgaggagcagtacaacagcacgtaccgtgtggtcagcgtcctcaccgtcctgcaccaggactggctgaatggcaaggagtacaagtgcaaggtctccaacaaagccctcccagcccccatcgagaaaaccatctccaaagccaaagggcagccccgagaaccacaggtgtacaccctgcccccatcccgtgatgagctgaccaagaaccaggtcagcctgacctgcctggtcaaaggcttctatcccagcgacatcgccgtggagtgggagagcaatgggcagccggagaacaactacaagaccacgcctcccgtgctggactccgacggctccttcttcctctacagcaagctcaccgtggacaagagccgttggcagcaggggaacgtcttctcatgctccgtgatgcatgaggctctgcacaaccactacacgcagaagagcctctccctgtctccgggtaaaggtggaggtggtggttctggtggtggtagcggtggtggtggatcccatccaattccagattcttctccattattacaattcgggggccaagtccggcagcggtacctctacacagatgatgcccagcagacagaagcccacctggagatcagggaggatgggacggtggggggcgctgctgaccagagccccgaaagtctcctgcagctgaaagccttgaagccgggagttattcaaatcttgggagtcaagacatccaggttcctgtgccagcggccagatggggccctgtatggatcgctccactttgaccctgaggcctgcagcttccgggagctgcttcttgaggacggatacaatgtttaccagtccgaagcccacggcctcccgctgcacctgccagggaacaagtccccacaccgggaccctgcaccccgaggaccagctcgcttcctgccactaccaggcctgccccccgcacccccggagccacccggaatcctggccccccagccccccgatgtgggctcctcggaccctctgagcatggtgtccccttcccagggccgaagccccagctacgcttcctaa

SEQ ID NO: 77 - protein, 424 aa, Artificial Sequence
  Synthetic Construct
MDKTHTCPPCPAPELLGGPSVFLFPPKPKDTLMISRTPEVTCVVVDVSHEDPEVKFNWYVDGVEVHNAKTKPREEQYNSTYRVVSVLTVLHQDWLNGKEYKCKVSNKALPAPIEKTISKAKGQPREPQVYTLPPSRDELTKNQVSLTCLVKGFYPSDIAVEWESNGQPENNYKTTPPVLDSDGSFFLYSKLTVDKSRWQQGNVFSCSVMHEALHNHYTQKSLSLSPGKGGGGGSGGGSGGGGSHPIPDSSPLLQFGGQVRQRYLYTDDAQQTEAHLEIREDGTVGGAADQSPESLLQLKALKPGVIQILGVKTSRFLCQRPDGALYGSLHFDPEACSFRELLLEDGYNVYQSEAHGLPLHLPGNKSPHRDPAPRGPARFLPLPGLPPAPPEPPGILAPQPPDVGSSDPLSMVSPSQGRSPSYAS

SEQ ID NO: 78 - DNA, 1275 bp, Artificial Sequence
  Fc-L15-P171E
  CDS (1)..(1275)
atggacaaaactcacacatgtccaccttgtccagctccggaactcctggggggaccgtcagtcttcctcttccccccaaaacccaaggacaccctcatgatctcccgtacccctgaggtcacatgcgtggtggtggacgtgagccacgaagaccctgaggtcaagttcaactggtacgtggacggcgtggaggtgcataatgccaagacaaagccgcgtgaggagcagtacaacagcacgtaccgtgtggtcagcgtcctcaccgtcctgcaccaggactggctgaatggcaaggagtacaagtgcaaggtctccaacaaagccctcccagcccccatcgagaaaaccatctccaaagccaaagggcagccccgagaaccacaggtgtacaccctgcccccatcccgtgatgagctgaccaagaaccaggtcagcctgacctgcctggtcaaaggcttctatcccagcgacatcgccgtggagtgggagagcaatgggcagccggagaacaactacaagaccacgcctcccgtgctggactccgacggctccttcttcctctacagcaagctcaccgtggacaagagccgttggcagcaggggaacgtcttctcatgctccgtgatgcatgaggctctgcacaaccactacacgcagaagagcctctccctgtctccgggtaaaggtggaggtggtggttctggtggtggtagcggtggtggtggatcccatccaattccagattcttctccattattacaattcgggggccaagtccggcagcggtacctctacacagatgatgcccagcagacagaagcccacctggagatcagggaggatgggacggtggggggcgctgctgaccagagccccgaaagtctcctgcagctgaaagccttgaagccgggagttattcaaatcttgggagtcaagacatccaggttcctgtgccagcggccagatggggccctgtatggatcgctccactttgaccctgaggcctgcagcttccgggagctgcttcttgaggacggatacaatgtttaccagtccgaagcccacggcctcccgctgcacctgccagggaacaagtccccacaccgggaccctgcaccccgaggaccagctcgcttcctgccactaccaggcctgccccccgcacccccggagccacccggaatcctggccccccagccccccgatgtgggctcctcggaccctctgagcatggtgggagaatcccagggccgaagccccagctacgcttcctaa

SEQ ID NO: 79 - protein, 424 aa, Artificial Sequence
  Synthetic Construct
MDKTHTCPPCPAPELLGGPSVFLFPPKPKDTLMISRTPEVTCVVVDVSHEDPEVKFNWYVDGVEVHNAKTKPREEQYNSTYRVVSVLTVLHQDWLNGKEYKCKVSNKALPAPIEKTISKAKGQPREPQVYTLPPSRDELTKNQVSLTCLVKGFYPSDIAVEWESNGQPENNYKTTPPVLDSDGSFFLYSKLTVDKSRWQQGNVFSCSVMHEALHNHYTQKSLSLSPGKGGGGGSGGGSGGGGSHPIPDSSPLLQFGGQVRQRYLYTDDAQQTEAHLEIREDGTVGGAADQSPESLLQLKALKPGVIQILGVKTSRFLCQRPDGALYGSLHFDPEACSFRELLLEDGYNVYQSEAHGLPLHLPGNKSPHRDPAPRGPARFLPLPGLPPAPPEPPGILAPQPPDVGSSDPLSMVGESQGRSPSYAS

SEQ ID NO: 80 - DNA, 1275 bp, Artificial Sequence
  Fc-L15-P171H
  CDS (1)..(1275)
atggacaaaactcacacatgtccaccttgtccagctccggaactcctggggggaccgtcagtcttcctcttccccccaaaacccaaggacaccctcatgatctcccgtacccctgaggtcacatgcgtggtggtggacgtgagccacgaagaccctgaggtcaagttcaactggtacgtggacggcgtggaggtgcataatgccaagacaaagccgcgtgaggagcagtacaacagcacgtaccgtgtggtcagcgtcctcaccgtcctgcaccaggactggctgaatggcaaggagtacaagtgcaaggtctccaacaaagccctcccagcccccatcgagaaaaccatctccaaagccaaagggcagccccgagaaccacaggtgtacaccctgcccccatcccgtgatgagctgaccaagaaccaggtcagcctgacctgcctggtcaaaggcttctatcccagcgacatcgccgtggagtgggagagcaatgggcagccggagaacaactacaagaccacgcctcccgtgctggactccgacggctccttcttcctctacagcaagctcaccgtggacaagagccgttggcagcaggggaacgtcttctcatgctccgtgatgcatgaggctctgcacaaccactacacgcagaagagcctctccctgtctccgggtaaaggtggaggtggtggttctggtggtggtagcggtggtggtggatcccatccaattccagattcttctccattattacaattcgggggccaagtccggcagcggtacctctacacagatgatgcccagcagacagaagcccacctggagatcagggaggatgggacggtggggggcgctgctgaccagagccccgaaagtctcctgcagctgaaagccttgaagccgggagttattcaaatcttgggagtcaagacatccaggttcctgtgccagcggccagatggggccctgtatggatcgctccactttgaccctgaggcctgcagcttccgggagctgcttcttgaggacggatacaatgtttaccagtccgaagcccacggcctcccgctgcacctgccagggaacaagtccccacaccgggaccctgcaccccgaggaccagctcgcttcctgccactaccaggcctgccccccgcacccccggagccacccggaatcctggccccccagccccccgatgtgggctcctcggaccctctgagcatggtgggacactcccagggccgaagccccagctacgcttcctaa

SEQ ID NO: 81 - protein, 424 aa, Artificial Sequence
  Synthetic Construct
MDKTHTCPPCPAPELLGGPSVFLFPPKPKDTLMISRTPEVTCVVVDVSHEDPEVKFNWYVDGVEVHNAKTKPREEQYNSTYRVVSVLTVLHQDWLNGKEYKCKVSNKALPAPIEKTISKAKGQPREPQVYTLPPSRDELTKNQVSLTCLVKGFYPSDIAVEWESNGQPENNYKTTPPVLDSDGSFFLYSKLTVDKSRWQQGNVFSCSVMHEALHNHYTQKSLSLSPGKGGGGGSGGGSGGGGSHPIPDSSPLLQFGGQVRQRYLYTDDAQQTEAHLEIREDGTVGGAADQSPESLLQLKALKPGVIQILGVKTSRFLCQRPDGALYGSLHFDPEACSFRELLLEDGYNVYQSEAHGLPLHLPGNKSPHRDPAPRGPARFLPLPGLPPAPPEPPGILAPQPPDVGSSDPLSMVGHSQGRSPSYAS

SEQ ID NO: 82 - DNA, 1275 bp, Artificial Sequence
  Fc-L15-P171Q
  CDS (1)..(1275)
atggacaaaactcacacatgtccaccttgtccagctccggaactcctggggggaccgtcagtcttcctcttccccccaaaacccaaggacaccctcatgatctcccgtacccctgaggtcacatgcgtggtggtggacgtgagccacgaagaccctgaggtcaagttcaactggtacgtggacggcgtggaggtgcataatgccaagacaaagccgcgtgaggagcagtacaacagcacgtaccgtgtggtcagcgtcctcaccgtcctgcaccaggactggctgaatggcaaggagtacaagtgcaaggtctccaacaaagccctcccagcccccatcgagaaaaccatctccaaagccaaagggcagccccgagaaccacaggtgtacaccctgcccccatcccgtgatgagctgaccaagaaccaggtcagcctgacctgcctggtcaaaggcttctatcccagcgacatcgccgtggagtgggagagcaatgggcagccggagaacaactacaagaccacgcctcccgtgctggactccgacggctccttcttcctctacagcaagctcaccgtggacaagagccgttggcagcaggggaacgtcttctcatgctccgtgatgcatgaggctctgcacaaccactacacgcagaagagcctctccctgtctccgggtaaaggtggaggtggtggttctggtggtggtagcggtggtggtggatcccatccaattccagattcttctccattattacaattcgggggccaagtccggcagcggtacctctacacagatgatgcccagcagacagaagcccacctggagatcagggaggatgggacggtggggggcgctgctgaccagagccccgaaagtctcctgcagctgaaagccttgaagccgggagttattcaaatcttgggagtcaagacatccaggttcctgtgccagcggccagatggggccctgtatggatcgctccactttgaccctgaggcctgcagcttccgggagctgcttcttgaggacggatacaatgtttaccagtccgaagcccacggcctcccgctgcacctgccagggaacaagtccccacaccgggaccctgcaccccgaggaccagctcgcttcctgccactaccaggcctgccccccgcacccccggagccacccggaatcctggccccccagccccccgatgtgggctcctcggaccctctgagcatggtgggacagtcccagggccgaagccccagctacgcttcctaa

SEQ ID NO: 83 - protein, 424 aa, Artificial Sequence
  Synthetic Construct
MDKTHTCPPCPAPELLGGPSVFLFPPKPKDTLMISRTPEVTCVVVDVSHEDPEVKFNWYVDGVEVHNAKTKPREEQYNSTYRVVSVLTVLHQDWLNGKEYKCKVSNKALPAPIEKTISKAKGQPREPQVYTLPPSRDELTKNQVSLTCLVKGFYPSDIAVEWESNGQPENNYKTTPPVLDSDGSFFLYSKLTVDKSRWQQGNVFSCSVMHEALHNHYTQKSLSLSPGKGGGGGSGGGSGGGGSHPIPDSSPLLQFGGQVRQRYLYTDDAQQTEAHLEIREDGTVGGAADQSPESLLQLKALKPGVIQILGVKTSRFLCQRPDGALYGSLHFDPEACSFRELLLEDGYNVYQSEAHGLPLHLPGNKSPHRDPAPRGPARFLPLPGLPPAPPEPPGILAPQPPDVGSSDPLSMVGQSQGRSPSYAS

SEQ ID NO: 84 - DNA, 1275 bp, Artificial Sequence
  Fc-L15-P171T
  CDS (1)..(1275)
atggacaaaactcacacatgtccaccttgtccagctccggaactcctggggggaccgtcagtcttcctcttccccccaaaacccaaggacaccctcatgatctcccgtacccctgaggtcacatgcgtggtggtggacgtgagccacgaagaccctgaggtcaagttcaactggtacgtggacggcgtggaggtgcataatgccaagacaaagccgcgtgaggagcagtacaacagcacgtaccgtgtggtcagcgtcctcaccgtcctgcaccaggactggctgaatggcaaggagtacaagtgcaaggtctccaacaaagccctcccagcccccatcgagaaaaccatctccaaagccaaagggcagccccgagaaccacaggtgtacaccctgcccccatcccgtgatgagctgaccaagaaccaggtcagcctgacctgcctggtcaaaggcttctatcccagcgacatcgccgtggagtgggagagcaatgggcagccggagaacaactacaagaccacgcctcccgtgctggactccgacggctccttcttcctctacagcaagctcaccgtggacaagagccgttggcagcaggggaacgtcttctcatgctccgtgatgcatgaggctctgcacaaccactacacgcagaagagcctctccctgtctccgggtaaaggtggaggtggtggttctggtggtggtagcggtggtggtggatcccatccaattccagattcttctccattattacaattcgggggccaagtccggcagcggtacctctacacagatgatgcccagcagacagaagcccacctggagatcagggaggatgggacggtggggggcgctgctgaccagagccccgaaagtctcctgcagctgaaagccttgaagccgggagttattcaaatcttgggagtcaagacatccaggttcctgtgccagcggccagatggggccctgtatggatcgctccactttgaccctgaggcctgcagcttccgggagctgcttcttgaggacggatacaatgtttaccagtccgaagcccacggcctcccgctgcacctgccagggaacaagtccccacaccgggaccctgcaccccgaggaccagctcgcttcctgccactaccaggcctgccccccgcacccccggagccacccggaatcctggccccccagccccccgatgtgggctcctcggaccctctgagcatggtgggaacttcccagggccgaagccccagctacgcttcctaa

SEQ ID NO: 85 - protein, 424 aa, Artificial Sequence
  Synthetic Construct
MDKTHTCPPCPAPELLGGPSVFLFPPKPKDTLMISRTPEVTCVVVDVSHEDPEVKFNWYVDGVEVHNAKTKPREEQYNSTYRVVSVLTVLHQDWLNGKEYKCKVSNKALPAPIEKTISKAKGQPREPQVYTLPPSRDELTKNQVSLTCLVKGFYPSDIAVEWESNGQPENNYKTTPPVLDSDGSFFLYSKLTVDKSRWQQGNVFSCSVMHEALHNHYTQKSLSLSPGKGGGGGSGGGSGGGGSHPIPDSSPLLQFGGQVRQRYLYTDDAQQTEAHLEIREDGTVGGAADQSPESLLQLKALKPGVIQILGVKTSRFLCQRPDGALYGSLHFDPEACSFRELLLEDGYNVYQSEAHGLPLHLPGNKSPHRDPAPRGPARFLPLPGLPPAPPEPPGILAPQPPDVGSSDPLSMVGTSQGRSPSYAS

SEQ ID NO: 86 - DNA, 1275 bp, Artificial Sequence
  Fc-L15-P171Y
  CDS (1)..(1275)
atggacaaaactcacacatgtccaccttgtccagctccggaactcctggggggaccgtcagtcttcctcttccccccaaaacccaaggacaccctcatgatctcccgtacccctgaggtcacatgcgtggtggtggacgtgagccacgaagaccctgaggtcaagttcaactggtacgtggacggcgtggaggtgcataatgccaagacaaagccgcgtgaggagcagtacaacagcacgtaccgtgtggtcagcgtcctcaccgtcctgcaccaggactggctgaatggcaaggagtacaagtgcaaggtctccaacaaagccctcccagcccccatcgagaaaaccatctccaaagccaaagggcagccccgagaaccacaggtgtacaccctgcccccatcccgtgatgagctgaccaagaaccaggtcagcctgacctgcctggtcaaaggcttctatcccagcgacatcgccgtggagtgggagagcaatgggcagccggagaacaactacaagaccacgcctcccgtgctggactccgacggctccttcttcctctacagcaagctcaccgtggacaagagccgttggcagcaggggaacgtcttctcatgctccgtgatgcatgaggctctgcacaaccactacacgcagaagagcctctccctgtctccgggtaaaggtggaggtggtggttctggtggtggtagcggtggtggtggatcccatccaattccagattcttctccattattacaattcgggggccaagtccggcagcggtacctctacacagatgatgcccagcagacagaagcccacctggagatcagggaggatgggacggtggggggcgctgctgaccagagccccgaaagtctcctgcagctgaaagccttgaagccgggagttattcaaatcttgggagtcaagacatccaggttcctgtgccagcggccagatggggccctgtatggatcgctccactttgaccctgaggcctgcagcttccgggagctgcttcttgaggacggatacaatgtttaccagtccgaagcccacggcctcccgctgcacctgccagggaacaagtccccacaccgggaccctgcaccccgaggaccagctcgcttcctgccactaccaggcctgccccccgcacccccggagccacccggaatcctggccccccagccccccgatgtgggctcctcggaccctctgagcatggtgggatactcccagggccgaagccccagctacgcttcctaa

SEQ ID NO: 87 - protein, 424 aa, Artificial Sequence
  Synthetic Construct
MDKTHTCPPCPAPELLGGPSVFLFPPKPKDTLMISRTPEVTCVVVDVSHEDPEVKFNWYVDGVEVHNAKTKPREEQYNSTYRVVSVLTVLHQDWLNGKEYKCKVSNKALPAPIEKTISKAKGQPREPQVYTLPPSRDELTKNQVSLTCLVKGFYPSDIAVEWESNGQPENNYKTTPPVLDSDGSFFLYSKLTVDKSRWQQGNVFSCSVMHEALHNHYTQKSLSLSPGKGGGGGSGGGSGGGGSHPIPDSSPLLQFGGQVRQRYLYTDDAQQTEAHLEIREDGTVGGAADQSPESLLQLKALKPGVIQILGVKTSRFLCQRPDGALYGSLHFDPEACSFRELLLEDGYNVYQSEAHGLPLHLPGNKSPHRDPAPRGPARFLPLPGLPPAPPEPPGILAPQPPDVGSSDPLSMVGYSQGRSPSYAS

SEQ ID NO: 88 - DNA, 1275 bp, Artificial Sequence
  Fc-L15-P171G
  CDS (1)..(1275)
atggacaaaactcacacatgtccaccttgtccagctccggaactcctggggggaccgtcagtcttcctcttccccccaaaacccaaggacaccctcatgatctcccgtacccctgaggtcacatgcgtggtggtggacgtgagccacgaagaccctgaggtcaagttcaactggtacgtggacggcgtggaggtgcataatgccaagacaaagccgcgtgaggagcagtacaacagcacgtaccgtgtggtcagcgtcctcaccgtcctgcaccaggactggctgaatggcaaggagtacaagtgcaaggtctccaacaaagccctcccagcccccatcgagaaaaccatctccaaagccaaagggcagccccgagaaccacaggtgtacaccctgcccccatcccgtgatgagctgaccaagaaccaggtcagcctgacctgcctggtcaaaggcttctatcccagcgacatcgccgtggagtgggagagcaatgggcagccggagaacaactacaagaccacgcctcccgtgctggactccgacggctccttcttcctctacagcaagctcaccgtggacaagagccgttggcagcaggggaacgtcttctcatgctccgtgatgcatgaggctctgcacaaccactacacgcagaagagcctctccctgtctccgggtaaaggtggaggtggtggttctggtggtggtagcggtggtggtggatcccatccaattccagattcttctccattattacaattcgggggccaagtccggcagcggtacctctacacagatgatgcccagcagacagaagcccacctggagatcagggaggatgggacggtggggggcgctgctgaccagagccccgaaagtctcctgcagctgaaagccttgaagccgggagttattcaaatcttgggagtcaagacatccaggttcctgtgccagcggccagatggggccctgtatggatcgctccactttgaccctgaggcctgcagcttccgggagctgcttcttgaggacggatacaatgtttaccagtccgaagcccacggcctcccgctgcacctgccagggaacaagtccccacaccgggaccctgcaccccgaggaccagctcgcttcctgccactaccaggcctgccccccgcacccccggagccacccggaatcctggccccccagccccccgatgtgggctcctcggaccctctgagcatggtgggaggttcccagggccgaagccccagctacgcttcctaa

SEQ ID NO: 89 - protein, 424 aa, Artificial Sequence
  Synthetic Construct
MDKTHTCPPCPAPELLGGPSVFLFPPKPKDTLMISRTPEVTCVVVDVSHEDPEVKFNWYVDGVEVHNAKTKPREEQYNSTYRVVSVLTVLHQDWLNGKEYKCKVSNKALPAPIEKTISKAKGQPREPQVYTLPPSRDELTKNQVSLTCLVKGFYPSDIAVEWESNGQPENNYKTTPPVLDSDGSFFLYSKLTVDKSRWQQGNVFSCSVMHEALHNHYTQKSLSLSPGKGGGGGSGGGSGGGGSHPIPDSSPLLQFGGQVRQRYLYTDDAQQTEAHLEIREDGTVGGAADQSPESLLQLKALKPGVIQILGVKTSRFLCQRPDGALYGSLHFDPEACSFRELLLEDGYNVYQSEAHGLPLHLPGNKSPHRDPAPRGPARFLPLPGLPPAPPEPPGILAPQPPDVGSSDPLSMVGGSQGRSPSYAS

SEQ ID NO: 90 - DNA, 1275 bp, Artificial Sequence
  Fc-L15-P171S
  CDS (1)..(1275)
atggacaaaactcacacatgtccaccttgtccagctccggaactcctggggggaccgtcagtcttcctcttccccccaaaacccaaggacaccctcatgatctcccgtacccctgaggtcacatgcgtggtggtggacgtgagccacgaagaccctgaggtcaagttcaactggtacgtggacggcgtggaggtgcataatgccaagacaaagccgcgtgaggagcagtacaacagcacgtaccgtgtggtcagcgtcctcaccgtcctgcaccaggactggctgaatggcaaggagtacaagtgcaaggtctccaacaaagccctcccagcccccatcgagaaaaccatctccaaagccaaagggcagccccgagaaccacaggtgtacaccctgcccccatcccgtgatgagctgaccaagaaccaggtcagcctgacctgcctggtcaaaggcttctatcccagcgacatcgccgtggagtgggagagcaatgggcagccggagaacaactacaagaccacgcctcccgtgctggactccgacggctccttcttcctctacagcaagctcaccgtggacaagagccgttggcagcaggggaacgtcttctcatgctccgtgatgcatgaggctctgcacaaccactacacgcagaagagcctctccctgtctccgggtaaaggtggaggtggtggttctggtggtggtagcggtggtggtggatcccatccaattccagattcttctccattattacaattcgggggccaagtccggcagcggtacctctacacagatgatgcccagcagacagaagcccacctggagatcagggaggatgggacggtggggggcgctgctgaccagagccccgaaagtctcctgcagctgaaagccttgaagccgggagttattcaaatcttgggagtcaagacatccaggttcctgtgccagcggccagatggggccctgtatggatcgctccactttgaccctgaggcctgcagcttccgggagctgcttcttgaggacggatacaatgtttaccagtccgaagcccacggcctcccgctgcacctgccagggaacaagtccccacaccgggaccctgcaccccgaggaccagctcgcttcctgccactaccaggcctgccccccgcacccccggagccacccggaatcctggccccccagccccccgatgtgggctcctcggaccctctgagcatggtgggatcttcccagggccgaagccccagctacgcttcctaa

SEQ ID NO: 91 - protein, 424 aa, Artificial Sequence
  Synthetic Construct
MDKTHTCPPCPAPELLGGPSVFLFPPKPKDTLMISRTPEVTCVVVDVSHEDPEVKFNWYVDGVEVHNAKTKPREEQYNSTYRVVSVLTVLHQDWLNGKEYKCKVSNKALPAPIEKTISKAKGQPREPQVYTLPPSRDELTKNQVSLTCLVKGFYPSDIAVEWESNGQPENNYKTTPPVLDSDGSFFLYSKLTVDKSRWQQGNVFSCSVMHEALHNHYTQKSLSLSPGKGGGGGSGGGSGGGGSHPIPDSSPLLQFGGQVRQRYLYTDDAQQTEAHLEIREDGTVGGAADQSPESLLQLKALKPGVIQILGVKTSRFLCQRPDGALYGSLHFDPEACSFRELLLEDGYNVYQSEAHGLPLHLPGNKSPHRDPAPRGPARFLPLPGLPPAPPEPPGILAPQPPDVGSSDPLSMVGSSQGRSPSYAS

SEQ ID NO: 92 - DNA, 1275 bp, Artificial Sequence
  Fc-L15-P171W
  CDS (1)..(1275)
atggacaaaactcacacatgtccaccttgtccagctccggaactcctggggggaccgtcagtcttcctcttccccccaaaacccaaggacaccctcatgatctcccgtacccctgaggtcacatgcgtggtggtggacgtgagccacgaagaccctgaggtcaagttcaactggtacgtggacggcgtggaggtgcataatgccaagacaaagccgcgtgaggagcagtacaacagcacgtaccgtgtggtcagcgtcctcaccgtcctgcaccaggactggctgaatggcaaggagtacaagtgcaaggtctccaacaaagccctcccagcccccatcgagaaaaccatctccaaagccaaagggcagccccgagaaccacaggtgtacaccctgcccccatcccgtgatgagctgaccaagaaccaggtcagcctgacctgcctggtcaaaggcttctatcccagcgacatcgccgtggagtgggagagcaatgggcagccggagaacaactacaagaccacgcctcccgtgctggactccgacggctccttcttcctctacagcaagctcaccgtggacaagagccgttggcagcaggggaacgtcttctcatgctccgtgatgcatgaggctctgcacaaccactacacgcagaagagcctctccctgtctccgggtaaaggtggaggtggtggttctggtggtggtagcggtggtggtggatcccatccaattccagattcttctccattattacaattcgggggccaagtccggcagcggtacctctacacagatgatgcccagcagacagaagcccacctggagatcagggaggatgggacggtggggggcgctgctgaccagagccccgaaagtctcctgcagctgaaagccttgaagccgggagttattcaaatcttgggagtcaagacatccaggttcctgtgccagcggccagatggggccctgtatggatcgctccactttgaccctgaggcctgcagcttccgggagctgcttcttgaggacggatacaatgtttaccagtccgaagcccacggcctcccgctgcacctgccagggaacaagtccccacaccgggaccctgcaccccgaggaccagctcgcttcctgccactaccaggcctgccccccgcacccccggagccacccggaatcctggccccccagccccccgatgtgggctcctcggaccctctgagcatggtgggatggtcccagggccgaagccccagctacgcttcctaa

SEQ ID NO: 93 - protein, 424 aa, Artificial Sequence
  Synthetic Construct
MDKTHTCPPCPAPELLGGPSVFLFPPKPKDTLMISRTPEVTCVVVDVSHEDPEVKFNWYVDGVEVHNAKTKPREEQYNSTYRVVSVLTVLHQDWLNGKEYKCKVSNKALPAPIEKTISKAKGQPREPQVYTLPPSRDELTKNQVSLTCLVKGFYPSDIAVEWESNGQPENNYKTTPPVLDSDGSFFLYSKLTVDKSRWQQGNVFSCSVMHEALHNHYTQKSLSLSPGKGGGGGSGGGSGGGGSHPIPDSSPLLQFGGQVRQRYLYTDDAQQTEAHLEIREDGTVGGAADQSPESLLQLKALKPGVIQILGVKTSRFLCQRPDGALYGSLHFDPEACSFRELLLEDGYNVYQSEAHGLPLHLPGNKSPHRDPAPRGPARFLPLPGLPPAPPEPPGILAPQPPDVGSSDPLSMVGWSQGRSPSYAS

SEQ ID NO: 94 - DNA, 1275 bp, Artificial Sequence
  Fc-L15-P171C
  CDS (1)..(1275)
atggacaaaactcacacatgtccaccttgtccagctccggaactcctggggggaccgtcagtcttcctcttccccccaaaacccaaggacaccctcatgatctcccgtacccctgaggtcacatgcgtggtggtggacgtgagccacgaagaccctgaggtcaagttcaactggtacgtggacggcgtggaggtgcataatgccaagacaaagccgcgtgaggagcagtacaacagcacgtaccgtgtggtcagcgtcctcaccgtcctgcaccaggactggctgaatggcaaggagtacaagtgcaaggtctccaacaaagccctcccagcccccatcgagaaaaccatctccaaagccaaagggcagccccgagaaccacaggtgtacaccctgcccccatcccgtgatgagctgaccaagaaccaggtcagcctgacctgcctggtcaaaggcttctatcccagcgacatcgccgtggagtgggagagcaatgggcagccggagaacaactacaagaccacgcctcccgtgctggactccgacggctccttcttcctctacagcaagctcaccgtggacaagagccgttggcagcaggggaacgtcttctcatgctccgtgatgcatgaggctctgcacaaccactacacgcagaagagcctctccctgtctccgggtaaaggtggaggtggtggttctggtggtggtagcggtggtggtggatcccatccaattccagattcttctccattattacaattcgggggccaagtccggcagcggtacctctacacagatgatgcccagcagacagaagcccacctggagatcagggaggatgggacggtggggggcgctgctgaccagagccccgaaagtctcctgcagctgaaagccttgaagccgggagttattcaaatcttgggagtcaagacatccaggttcctgtgccagcggccagatggggccctgtatggatcgctccactttgaccctgaggcctgcagcttccgggagctgcttcttgaggacggatacaatgtttaccagtccgaagcccacggcctcccgctgcacctgccagggaacaagtccccacaccgggaccctgcaccccgaggaccagctcgcttcctgccactaccaggcctgccccccgcacccccggagccacccggaatcctggccccccagccccccgatgtgggctcctcggaccctctgagcatggtgggatgctcccagggccgaagccccagctacgcttcctaa

SEQ ID NO: 95 - protein, 424 aa, Artificial Sequence
  Synthetic Construct
MDKTHTCPPCPAPELLGGPSVFLFPPKPKDTLMISRTPEVTCVVVDVSHEDPEVKFNWYVDGVEVHNAKTKPREEQYNSTYRVVSVLTVLHQDWLNGKEYKCKVSNKALPAPIEKTISKAKGQPREPQVYTLPPSRDELTKNQVSLTCLVKGFYPSDIAVEWESNGQPENNYKTTPPVLDSDGSFFLYSKLTVDKSRWQQGNVFSCSVMHEALHNHYTQKSLSLSPGKGGGGGSGGGSGGGGSHPIPDSSPLLQFGGQVRQRYLYTDDAQQTEAHLEIREDGTVGGAADQSPESLLQLKALKPGVIQILGVKTSRFLCQRPDGALYGSLHFDPEACSFRELLLEDGYNVYQSEAHGLPLHLPGNKSPHRDPAPRGPARFLPLPGLPPAPPEPPGILAPQPPDVGSSDPLSMVGCSQGRSPSYAS

SEQ ID NO: 96 - DNA, 1275 bp, Artificial Sequence
  Fc-L15-A45K G170E
  CDS (1)..(1275)
atggacaaaactcacacatgtccaccttgtccagctccggaactcctggggggaccgtcagtcttcctcttccccccaaaacccaaggacaccctcatgatctcccgtacccctgaggtcacatgcgtggtggtggacgtgagccacgaagaccctgaggtcaagttcaactggtacgtggacggcgtggaggtgcataatgccaagacaaagccgcgtgaggagcagtacaacagcacgtaccgtgtggtcagcgtcctcaccgtcctgcaccaggactggctgaatggcaaggagtacaagtgcaaggtctccaacaaagccctcccagcccccatcgagaaaaccatctccaaagccaaagggcagccccgagaaccacaggtgtacaccctgcccccatcccgtgatgagctgaccaagaaccaggtcagcctgacctgcctggtcaaaggcttctatcccagcgacatcgccgtggagtgggagagcaatgggcagccggagaacaactacaagaccacgcctcccgtgctggactccgacggctccttcttcctctacagcaagctcaccgtggacaagagccgttggcagcaggggaacgtcttctcatgctccgtgatgcatgaggctctgcacaaccactacacgcagaagagcctctccctgtctccgggtaaaggtggaggtggtggttctggtggtggtagcggtggtggtggatcccatccaattccagattcttctccattattacaattcgggggccaagtccggcagcggtacctctacacagatgatgcccagcagacagaagcccacctggagatcagggaggatgggacggtggggggcgctaaagaccagagccccgaaagtctcctgcagctgaaagccttgaagccgggagttattcaaatcttgggagtcaagacatccaggttcctgtgccagcggccagatggggccctgtatggatcgctccactttgaccctgaggcctgcagcttccgggagctgcttcttgaggacggatacaatgtttaccagtccgaagcccacggcctcccgctgcacctgccagggaacaagtccccacaccgggaccctgcaccccgaggaccagctcgcttcctgccactaccaggcctgccccccgcacccccggagccacccggaatcctggccccccagccccccgatgtgggctcctcggaccctctgagcatggtggaaccttcccagggccgaagccccagctacgcttcctaa

SEQ ID NO: 97 - protein, 424 aa, Artificial Sequence
  Synthetic Construct
MDKTHTCPPCPAPELLGGPSVFLFPPKPKDTLMISRTPEVTCVVVDVSHEDPEVKFNWYVDGVEVHNAKTKPREEQYNSTYRVVSVLTVLHQDWLNGKEYKCKVSNKALPAPIEKTISKAKGQPREPQVYTLPPSRDELTKNQVSLTCLVKGFYPSDIAVEWESNGQPENNYKTTPPVLDSDGSFFLYSKLTVDKSRWQQGNVFSCSVMHEALHNHYTQKSLSLSPGKGGGGGSGGGSGGGGSHPIPDSSPLLQFGGQVRQRYLYTDDAQQTEAHLEIREDGTVGGAKDQSPESLLQLKALKPGVIQILGVKTSRFLCQRPDGALYGSLHFDPEACSFRELLLEDGYNVYQSEAHGLPLHLPGNKSPHRDPAPRGPARFLPLPGLPPAPPEPPGILAPQPPDVGSSDPLSMVEPSQGRSPSYAS

SEQ ID NO: 98 - DNA, 549 bp, Artificial Sequence
  FGF21 A45K
  CDS (1)..(549)
atgcatccaattccagattcttctccattattacaattcgggggccaagtccggcagcggtacctctacacagatgatgcccagcagacagaagcccacctggagatcagggaggatgggacggtggggggcgctaaagaccagagccccgaaagtctcctgcagctgaaagccttgaagccgggagttattcaaatcttgggagtcaagacatccaggttcctgtgccagcggccagatggggccctgtatggatcgctccactttgaccctgaggcctgcagcttccgggagctgcttcttgaggacggatacaatgtttaccagtccgaagcccacggcctcccgctgcacctgccagggaacaagtccccacaccgggaccctgcaccccgaggaccagctcgcttcctgccactaccaggcctgccccccgcacccccggagccacccggaatcctggccccccagccccccgatgtgggctcctcggaccctctgagcatggtgggaccttcccagggccgaagccccagctacgcttcctaa

SEQ ID NO: 99 - protein, 182 aa, Artificial Sequence
  Synthetic Construct
MHPIPDSSPLLQFGGQVRQRYLYTDDAQQTEAHLEIREDGTVGGAKDQSPESLLQLKALKPGVIQILGVKTSRFLCQRPDGALYGSLHFDPEACSFRELLLEDGYNVYQSEAHGLPLHLPGNKSPHRDPAPRGPARFLPLPGLPPAPPEPPGILAPQPPDVGSSDPLSMVGPSQGRSPSYAS

SEQ ID NO: 100 - DNA, 1260 bp, Artificial Sequence
  Fc-L15-FGF21 6-181 G170E
  CDS (1)..(1260)
atggacaaaactcacacatgtccaccttgtccagctccggaactcctggggggaccgtcagtcttcctcttccccccaaaacccaaggacaccctcatgatctcccgtacccctgaggtcacatgcgtggtggtggacgtgagccacgaagaccctgaggtcaagttcaactggtacgtggacggcgtggaggtgcataatgccaagacaaagccgcgtgaggagcagtacaacagcacgtaccgtgtggtcagcgtcctcaccgtcctgcaccaggactggctgaatggcaaggagtacaagtgcaaggtctccaacaaagccctcccagcccccatcgagaaaaccatctccaaagccaaagggcagccccgagaaccacaggtgtacaccctgcccccatcccgtgatgagctgaccaagaaccaggtcagcctgacctgcctggtcaaaggcttctatcccagcgacatcgccgtggagtgggagagcaatgggcagccggagaacaactacaagaccacgcctcccgtgctggactccgacggctccttcttcctctacagcaagctcaccgtggacaagagccgttggcagcaggggaacgtcttctcatgctccgtgatgcatgaggctctgcacaaccactacacgcagaagagcctctccctgtctccgggtaaaggtggaggtggtggttctggtggtggtagcggtggtggtggatcctcttctccattattacaattcggtggtcaagtccggcagcggtacctctacacagatgatgcccagcagacagaagcccacctggagatcagggaggatgggacggtggggggcgctgctgaccagagccccgaaagtctcctgcagctgaaagccttgaagccgggagttattcaaatcttgggagtcaagacatccaggttcctgtgccagcggccagatggggccctgtatggatcgctccactttgaccctgaggcctgcagcttccgggagctgcttcttgaggacggatacaatgtttaccagtccgaagcccacggcctcccgctgcacctgccagggaacaagtccccacaccgggaccctgcaccccgaggaccagctcgcttcctgccactaccaggcctgccccccgcacccccggagccacccggaatcctggccccccagccccccgatgtgggctcctcggaccctctgagcatggtggaaccttcccagggccgaagccccagctacgcttcctaa

SEQ ID NO: 101 - protein, 419 aa, Artificial Sequence
  Synthetic Construct
MDKTHTCPPCPAPELLGGPSVFLFPPKPKDTLMISRTPEVTCVVVDVSHEDPEVKFNWYVDGVEVHNAKTKPREEQYNSTYRVVSVLTVLHQDWLNGKEYKCKVSNKALPAPIEKTISKAKGQPREPQVYTLPPSRDELTKNQVSLTCLVKGFYPSDIAVEWESNGQPENNYKTTPPVLDSDGSFFLYSKLTVDKSRWQQGNVFSCSVMHEALHNHYTQKSLSLSPGKGGGGGSGGGSGGGGSSSPLLQFGGQVRQRYLYTDDAQQTEAHLEIREDGTVGGAADQSPESLLQLKALKPGVIQILGVKTSRFLCQRPDGALYGSLHFDPEACSFRELLLEDGYNVYQSEAHGLPLHLPGNKSPHRDPAPRGPARFLPLPGLPPAPPEPPGILAPQPPDVGSSDPLSMVEPSQGRSPSYAS

SEQ ID NO: 102 - DNA, 1275 bp, Artificial Sequence
  Fc-L15-A45K P171G
  CDS (1)..(1275)
atggacaaaactcacacatgtccaccttgtccagctccggaactcctggggggaccgtcagtcttcctcttccccccaaaacccaaggacaccctcatgatctcccgtacccctgaggtcacatgcgtggtggtggacgtgagccacgaagaccctgaggtcaagttcaactggtacgtggacggcgtggaggtgcataatgccaagacaaagccgcgtgaggagcagtacaacagcacgtaccgtgtggtcagcgtcctcaccgtcctgcaccaggactggctgaatggcaaggagtacaagtgcaaggtctccaacaaagccctcccagcccccatcgagaaaaccatctccaaagccaaagggcagccccgagaaccacaggtgtacaccctgcccccatcccgtgatgagctgaccaagaaccaggtcagcctgacctgcctggtcaaaggcttctatcccagcgacatcgccgtggagtgggagagcaatgggcagccggagaacaactacaagaccacgcctcccgtgctggactccgacggctccttcttcctctacagcaagctcaccgtggacaagagccgttggcagcaggggaacgtcttctcatgctccgtgatgcatgaggctctgcacaaccactacacgcagaagagcctctccctgtctccgggtaaaggtggaggtggtggttctggtggtggtagcggtggtggtggatcccatccaattccagattcttctccattattacaattcgggggccaagtccggcagcggtacctctacacagatgatgcccagcagacagaagcccacctggagatcagggaggatgggacggtggggggcgctaaagaccagagccccgaaagtctcctgcagctgaaagccttgaagccgggagttattcaaatcttgggagtcaagacatccaggttcctgtgccagcggccagatggggccctgtatggatcgctccactttgaccctgaggcctgcagcttccgggagctgcttcttgaggacggatacaatgtttaccagtccgaagcccacggcctcccgctgcacctgccagggaacaagtccccacaccgggaccctgcaccccgaggaccagctcgcttcctgccactaccaggcctgccccccgcacccccggagccacccggaatcctggccccccagccccccgatgtgggctcctcggaccctctgagcatggtgggaggttcccagggccgaagccccagctacgcttcctaa

SEQ ID NO: 103 - protein, 424 aa, Artificial Sequence
  Synthetic Construct
MDKTHTCPPCPAPELLGGPSVFLFPPKPKDTLMISRTPEVTCVVVDVSHEDPEVKFNWYVDGVEVHNAKTKPREEQYNSTYRVVSVLTVLHQDWLNGKEYKCKVSNKALPAPIEKTISKAKGQPREPQVYTLPPSRDELTKNQVSLTCLVKGFYPSDIAVEWESNGQPENNYKTTPPVLDSDGSFFLYSKLTVDKSRWQQGNVFSCSVMHEALHNHYTQKSLSLSPGKGGGGGSGGGSGGGGSHPIPDSSPLLQFGGQVRQRYLYTDDAQQTEAHLEIREDGTVGGAKDQSPESLLQLKALKPGVIQILGVKTSRFLCQRPDGALYGSLHFDPEACSFRELLLEDGYNVYQSEAHGLPLHLPGNKSPHRDPAPRGPARFLPLPGLPPAPPEPPGILAPQPPDVGSSDPLSMVGGSQGRSPSYAS

SEQ ID NO: 104 - DNA, 1320 bp, Artificial Sequence
  FGF21-(G3)-Fc; 28 AA signal sequence removed during processing
  CDS (1)..(1320)
atggactcggacgagaccgggttcgagcactcaggactgtgggtttctgtgctggctggtcttctgctgggagcctgccaggcacaccccatccctgactccagtcctctcctgcaattcgggggccaagtccggcagcggtacctctacacagatgatgcccagcagacagaagcccacctggagatcagggaggatgggacggtggggggcgctgctgaccagagccccgaaagtctcctgcagctgaaagccttgaagccgggagttattcaaatcttgggagtcaagacatccaggttcctgtgccagcggccagatggggccctgtatggatcgctccactttgaccctgaggcctgcagcttccgggagctgcttcttgaggacggatacaatgtttaccagtccgaagcccacggcctcccgctgcacctgccagggaacaagtccccacaccgggaccctgcaccccgaggaccagctcgcttcctgccactaccaggcctgccacccgcacccccggagccacccggaatcctggccccccagccccccgatgtgggctcctcggaccctctgagcatggtgggaccttcccagggccgaagccccagctacgcttccggtggaggtgacaaaactcacacatgcccaccgtgcccagcacctgaactcctggggggaccgtcagtcttcctcttccccccaaaacccaaggacaccctcatgatctcccggacccctgaggtcacatgcgtggtggtggacgtgagccacgaagaccctgaggtcaagttcaactggtacgtggacggcgtggaggtgcataatgccaagacaaagccgcgggaggagcagtacaacagcacgtaccgtgtggtcagcgtcctcaccgtcctgcaccaggactggctgaatggcaaggagtacaagtgcaaggtctccaacaaagccctcccagcccccatcgagaaaaccatctccaaagccaaagggcagccccgagaaccacaggtgtacaccctgcccccatcccgggatgagctgaccaagaaccaggtcagcctgacctgcctggtcaaaggcttctatcccagcgacatcgccgtggagtgggagagcaatgggcagccggagaacaactacaagaccacgcctcccgtgctggactccgacggctccttcttcctctatagcaagctcaccgtggacaagagcaggtggcagcaggggaacgtcttctcatgctccgtgatgcatgaggctctgcacaaccactacacgcagaagagcctctccctgtctccgggtaaatga

SEQ ID NO: 105 - protein, 439 aa, Artificial Sequence
  Synthetic Construct
MDSDETGFEHSGLWVSVLAGLLLGACQAHPIPDSSPLLQFGGQVRQRYLYTDDAQQTEAHLEIREDGTVGGAADQSPESLLQLKALKPGVIQILGVKTSRFLCQRPDGALYGSLHFDPEACSFRELLLEDGYNVYQSEAHGLPLHLPGNKSPHRDPAPRGPARFLPLPGLPPAPPEPPGILAPQPPDVGSSDPLSMVGPSQGRSPSYASGGGDKTHTCPPCPAPELLGGPSVFLFPPKPKDTLMISRTPEVTCVVVDVSHEDPEVKFNWYVDGVEVHNAKTKPREEQYNSTYRVVSVLTVLHQDWLNGKEYKCKVSNKALPAPIEKTISKAKGQPREPQVYTLPPSRDELTKNQVSLTCLVKGFYPSDIAVEWESNGQPENNYKTTPPVLDSDGSFFLYSKLTVDKSRWQQGNVFSCSVMHEALHNHYTQKSLSLSPGK

SEQ ID NO: 106 - DNA, 1245 bp, Artificial Sequence
  Fc-G5-FGF21
  CDS (1)..(1245)
atggacaaaactcacacatgtccaccttgtccagctccggaactcctggggggaccgtcagtcttcctcttccccccaaaacccaaggacaccctcatgatctcccggacccctgaggtcacatgcgtggtggtggacgtgagccacgaagaccctgaggtcaagttcaactggtacgtggacggcgtggaggtgcataatgccaagacaaagccgcgggaggagcagtacaacagcacgtaccgtgtggtcagcgtcctcaccgtcctgcaccaggactggctgaatggcaaggagtacaagtgcaaggtctccaacaaagccctcccagcccccatcgagaaaaccatctccaaagccaaagggcagccccgagaaccacaggtgtacaccctgcccccatcccgggatgagctgaccaagaaccaggtcagcctgacctgcctggtcaaaggcttctatcccagcgacatcgccgtggagtgggagagcaatgggcagccggagaacaactacaagaccacgcctcccgtgctggactccgacggctccttcttcctctacagcaagctcaccgtggacaagagcaggtggcagcaggggaacgtcttctcatgctccgtgatgcatgaggctctgcacaaccactacacgcagaagagcctctccctgtctccgggtaaaggtggcggagggggtcatccaattccagattcttctccattattacaattcgggggccaagtccggcagcggtacctctacacagatgatgcccagcagacagaagcccacctggagatcagggaggatgggacggtggggggcgctgctgaccagagccccgaaagtctcctgcagctgaaagccttgaagccgggagttattcaaatcttgggagtcaagacatccaggttcctgtgccagcggccagatggggccctgtatggatcgctccactttgaccctgaggcctgcagcttccgggagctgcttcttgaggacggatacaatgtttaccagtccgaagcccacggcctcccgctgcacctgccagggaacaagtccccacaccgggaccctgcaccccgaggaccagctcgcttcctgccactaccaggcctgccccccgcacccccggagccacccggaatcctggccccccagccccccgatgtgggctcctcggaccctctgagcatggtgggaccttcccagggccgaagccccagctacgcttcctaa

SEQ ID NO: 107 - protein, 414 aa, Artificial Sequence
  Synthetic Construct
MDKTHTCPPCPAPELLGGPSVFLFPPKPKDTLMISRTPEVTCVVVDVSHEDPEVKFNWYVDGVEVHNAKTKPREEQYNSTYRVVSVLTVLHQDWLNGKEYKCKVSNKALPAPIEKTISKAKGQPREPQVYTLPPSRDELTKNQVSLTCLVKGFYPSDIAVEWESNGQPENNYKTTPPVLDSDGSFFLYSKLTVDKSRWQQGNVFSCSVMHEALHNHYTQKSLSLSPGKGGGGGHPIPDSSPLLQFGGQVRQRYLYTDDAQQTEAHLEIREDGTVGGAADQSPESLLQLKALKPGVIQILGVKTSRFLCQRPDGALYGSLHFDPEACSFRELLLEDGYNVYQSEAHGLPLHLPGNKSPHRDPAPRGPARFLPLPGLPPAPPEPPGILAPQPPDVGSSDPLSMVGPSQGRSPSYAS

SEQ ID NO: 108 - DNA, 549 bp, Artificial Sequence
  FGF21 L99R
  CDS (1)..(549)
atgcatccaattccagattcttctccattattacaattcgggggccaagtccggcagcggtacctctacacagatgatgcccagcagacagaagcccacctggagatcagggaggatgggacggtggggggcgctgctgaccagagccccgaaagtctcctgcagctgaaagccttgaagccgggagttattcaaatcttgggagtcaagacatccaggttcctgtgccagcggccagatggggccctgtatggatcgctccactttgaccctgaggcctgcagcttccgggagctgcgtcttgaggacggatacaatgtttaccagtccgaagcccacggcctcccgctgcacctgccagggaacaagtccccacaccgggaccctgcaccccgaggaccagctcgcttcctgccactaccaggcctgccccccgcacccccggagccacccggaatcctggccccccagccccccgatgtgggctcctcggaccctctgagcatggtgggaccttcccagggccgaagccccagctacgcttcctaa

SEQ ID NO: 109 - protein, 182 aa, Artificial Sequence
  Synthetic Construct
MHPIPDSSPLLQFGGQVRQRYLYTDDAQQTEAHLEIREDGTVGGAADQSPESLLQLKALKPGVIQILGVKTSRFLCQRPDGALYGSLHFDPEACSFRELRLEDGYNVYQSEAHGLPLHLPGNKSPHRDPAPRGPARFLPLPGLPPAPPEPPGILAPQPPDVGSSDPLSMVGPSQGRSPSYAS

SEQ ID NO: 110 - DNA, 549 bp, Artificial Sequence
  FGF21 L99D
  CDS (1)..(549)
atgcatccaattccagattcttctccattattacaattcgggggccaagtccggcagcggtacctctacacagatgatgcccagcagacagaagcccacctggagatcagggaggatgggacggtggggggcgctgctgaccagagccccgaaagtctcctgcagctgaaagccttgaagccgggagttattcaaatcttgggagtcaagacatccaggttcctgtgccagcggccagatggggccctgtatggatcgctccactttgaccctgaggcctgcagcttccgggagctggaccttgaggacggatacaatgtttaccagtccgaagcccacggcctcccgctgcacctgccagggaacaagtccccacaccgggaccctgcaccccgaggaccagctcgcttcctgccactaccaggcctgccccccgcacccccggagccacccggaatcctggccccccagccccccgatgtgggctcctcggaccctctgagcatggtgggaccttcccagggccgaagccccagctacgcttcctaa

SEQ ID NO: 111 - protein, 182 aa, Artificial Sequence
  Synthetic Construct
MHPIPDSSPLLQFGGQVRQRYLYTDDAQQTEAHLEIREDGTVGGAADQSPESLLQLKALKPGVIQILGVKTSRFLCQRPDGALYGSLHFDPEACSFRELDLEDGYNVYQSEAHGLPLHLPGNKSPHRDPAPRGPARFLPLPGLPPAPPEPPGILAPQPPDVGSSDPLSMVGPSQGRSPSYAS

SEQ ID NO: 112 - DNA, 549 bp, Artificial Sequence
  FGF21 A111T
  CDS (1)..(549)
atgcatccaattccagattcttctccattattacaattcgggggccaagtccggcagcggtacctctacacagatgatgcccagcagacagaagcccacctggagatcagggaggatgggacggtggggggcgctgctgaccagagccccgaaagtctcctgcagctgaaagccttgaagccgggagttattcaaatcttgggagtcaagacatccaggttcctgtgccagcggccagatggggccctgtatggatcgctccactttgaccctgaggcctgcagcttccgggagctgcttcttgaggacggatacaatgtttaccagtccgaaacccacggcctcccgctgcacctgccagggaacaagtccccacaccgggaccctgcaccccgaggaccagctcgcttcctgccactaccaggcctgccccccgcacccccggagccacccggaatcctggccccccagccccccgatgtgggctcctcggaccctctgagcatggtgggaccttcccagggccgaagccccagctacgcttcctaa

SEQ ID NO: 113 - protein, 182 aa, Artificial Sequence
  Synthetic Construct
MHPIPDSSPLLQFGGQVRQRYLYTDDAQQTEAHLEIREDGTVGGAADQSPESLLQLKALKPGVIQILGVKTSRFLCQRPDGALYGSLHFDPEACSFRELLLEDGYNVYQSETHGLPLHLPGNKSPHRDPAPRGPARFLPLPGLPPAPPEPPGILAPQPPDVGSSDPLSMVGPSQGRSPSYAS

SEQ ID NO: 114 - DNA, 549 bp, Artificial Sequence
  FGF21 A129D
  CDS (1)..(549)
atgcatccaattccagattcttctccattattacaattcgggggccaagtccggcagcggtacctctacacagatgatgcccagcagacagaagcccacctggagatcagggaggatgggacggtggggggcgctgctgaccagagccccgaaagtctcctgcagctgaaagccttgaagccgggagttattcaaatcttgggagtcaagacatccaggttcctgtgccagcggccagatggggccctgtatggatcgctccactttgaccctgaggcctgcagcttccgggagctgcttcttgaggacggatacaatgtttaccagtccgaagcccacggcctcccgctgcacctgccagggaacaagtccccacaccgggaccctgacccccgaggaccagctcgcttcctgccactaccaggcctgccccccgcacccccggagccacccggaatcctggccccccagccccccgatgtgggctcctcggaccctctgagcatggtgggaccttcccagggccgaagccccagctacgcttcctaa

SEQ ID NO: 115 - protein, 182 aa, Artificial Sequence
  Synthetic Construct
MHPIPDSSPLLQFGGQVRQRYLYTDDAQQTEAHLEIREDGTVGGAADQSPESLLQLKALKPGVIQILGVKTSRFLCQRPDGALYGSLHFDPEACSFRELLLEDGYNVYQSEAHGLPLHLPGNKSPHRDPDPRGPARFLPLPGLPPAPPEPPGILAPQPPDVGSSDPLSMVGPSQGRSPSYAS

SEQ ID NO: 116 - DNA, 549 bp, Artificial Sequence
  FGF21 A129Q
  CDS (1)..(549)
atgcatccaattccagattcttctccattattacaattcgggggccaagtccggcagcggtacctctacacagatgatgcccagcagacagaagcccacctggagatcagggaggatgggacggtggggggcgctgctgaccagagccccgaaagtctcctgcagctgaaagccttgaagccgggagttattcaaatcttgggagtcaagacatccaggttcctgtgccagcggccagatggggccctgtatggatcgctccactttgaccctgaggcctgcagcttccgggagctgcttcttgaggacggatacaatgtttaccagtccgaagcccacggcctcccgctgcacctgccagggaacaagtccccacaccgggaccctcagccccgaggaccagctcgcttcctgccactaccaggcctgccccccgcacccccggagccacccggaatcctggccccccagccccccgatgtgggctcctcggaccctctgagcatggtgggaccttcccagggccgaagccccagctacgcttcctaa

SEQ ID NO: 117 - protein, 182 aa, Artificial Sequence
  Synthetic Construct
MHPIPDSSPLLQFGGQVRQRYLYTDDAQQTEAHLEIREDGTVGGAADQSPESLLQLKALKPGVIQILGVKTSRFLCQRPDGALYGSLHFDPEACSFRELLLEDGYNVYQSEAHGLPLHLPGNKSPHRDPQPRGPARFLPLPGLPPAPPEPPGILAPQPPDVGSSDPLSMVGPSQGRSPSYAS

SEQ ID NO: 118 - DNA, 549 bp, Artificial Sequence
  FGF21 A134K
  CDS (1)..(549)
atgcatccaattccagattcttctccattattacaattcgggggccaagtccggcagcggtacctctacacagatgatgcccagcagacagaagcccacctggagatcagggaggatgggacggtggggggcgctgctgaccagagccccgaaagtctcctgcagctgaaagccttgaagccgggagttattcaaatcttgggagtcaagacatccaggttcctgtgccagcggccagatggggccctgtatggatcgctccactttgaccctgaggcctgcagcttccgggagctgcttcttgaggacggatacaatgtttaccagtccgaagcccacggcctcccgctgcacctgccagggaacaagtccccacaccgggaccctgcaccccgaggaccaaaacgcttcctgccactaccaggcctgccccccgcacccccggagccacccggaatcctggccccccagccccccgatgtgggctcctcggaccctctgagcatggtgggaccttcccagggccgaagccccagctacgcttcctaa

SEQ ID NO: 119 - protein, 182 aa, Artificial Sequence
  Synthetic Construct
MHPIPDSSPLLQFGGQVRQRYLYTDDAQQTEAHLEIREDGTVGGAADQSPESLLQLKALKPGVIQILGVKTSRFLCQRPDGALYGSLHFDPEACSFRELLLEDGYNVYQSEAHGLPLHLPGNKSPHRDPAPRGPKRFLPLPGLPPAPPEPPGILAPQPPDVGSSDPLSMVGPSQGRSPSYAS

SEQ ID NO: 120 - DNA, 549 bp, Artificial Sequence
  FGF21 A134Y
  CDS (1)..(549)
atgcatccaattccagattcttctccattattacaattcgggggccaagtccggcagcggtacctctacacagatgatgcccagcagacagaagcccacctggagatcagggaggatgggacggtggggggcgctgctgaccagagccccgaaagtctcctgcagctgaaagccttgaagccgggagttattcaaatcttgggagtcaagacatccaggttcctgtgccagcggccagatggggccctgtatggatcgctccactttgaccctgaggcctgcagcttccgggagctgcttcttgaggacggatacaatgtttaccagtccgaagcccacggcctcccgctgcacctgccagggaacaagtccccacaccgggaccctgcaccccgaggaccatatcgcttcctgccactaccaggcctgccccccgcacccccggagccacccggaatcctggccccccagccccccgatgtgggctcctcggaccctctgagcatggtgggaccttcccagggccgaagccccagctacgcttcctaa

SEQ ID NO: 121 - protein, 182 aa, Artificial Sequence
  Synthetic Construct
MHPIPDSSPLLQFGGQVRQRYLYTDDAQQTEAHLEIREDGTVGGAADQSPESLLQLKALKPGVIQILGVKTSRFLCQRPDGALYGSLHFDPEACSFRELLLEDGYNVYQSEAHGLPLHLPGNKSPHRDPAPRGPYRFLPLPGLPPAPPEPPGILAPQPPDVGSSDPLSMVGPSQGRSPSYAS

SEQ ID NO: 122 - DNA, 549 bp, Artificial Sequence
  FGF21 A134E
  CDS (1)..(549)
atgcatccaattccagattcttctccattattacaattcgggggccaagtccggcagcggtacctctacacagatgatgcccagcagacagaagcccacctggagatcagggaggatgggacggtggggggcgctgctgaccagagccccgaaagtctcctgcagctgaaagccttgaagccgggagttattcaaatcttgggagtcaagacatccaggttcctgtgccagcggccagatggggccctgtatggatcgctccactttgaccctgaggcctgcagcttccgggagctgcttcttgaggacggatacaatgtttaccagtccgaagcccacggcctcccgctgcacctgccagggaacaagtccccacaccgggaccctgcaccccgaggaccagaacgcttcctgccactaccaggcctgccccccgcacccccggagccacccggaatcctggccccccagccccccgatgtgggctcctcggaccctctgagcatggtgggaccttcccagggccgaagccccagctacgcttcctaa

SEQ ID NO: 123 - protein, 182 aa, Artificial Sequence
  Synthetic Construct
MHPIPDSSPLLQFGGQVRQRYLYTDDAQQTEAHLEIREDGTVGGAADQSPESLLQLKALKPGVIQILGVKTSRFLCQRPDGALYGSLHFDPEACSFRELLLEDGYNVYQSEAHGLPLHLPGNKSPHRDPAPRGPERFLPLPGLPPAPPEPPGILAPQPPDVGSSDPLSMVGPSQGRSPSYAS

SEQ ID NO: 124 - DNA, 549 bp, Artificial Sequence
  FGF21 A129K
  CDS (1)..(549)
atgcatccaattccagattcttctccattattacaattcgggggccaagtccggcagcggtacctctacacagatgatgcccagcagacagaagcccacctggagatcagggaggatgggacggtggggggcgctgctgaccagagccccgaaagtctcctgcagctgaaagccttgaagccgggagttattcaaatcttgggagtcaagacatccaggttcctgtgccagcggccagatggggccctgtatggatcgctccactttgaccctgaggcctgcagcttccgggagctgcttcttgaggacggatacaatgtttaccagtccgaagcccacggcctcccgctgcacctgccagggaacaagtccccacaccgggaccctaaaccccgaggaccagctcgcttcctgccactaccaggcctgccccccgcacccccggagccacccggaatcctggccccccagccccccgatgtgggctcctcggaccctctgagcatggtgggaccttcccagggccgaagccccagctacgcttcctaa

SEQ ID NO: 125 - protein, 182 aa, Artificial Sequence
  Synthetic Construct
MHPIPDSSPLLQFGGQVRQRYLYTDDAQQTEAHLEIREDGTVGGAADQSPESLLQLKALKPGVIQILGVKTSRFLCQRPDGALYGSLHFDPEACSFRELLLEDGYNVYQSEAHGLPLHLPGNKSPHRDPKPRGPARFLPLPGLPPAPPEPPGILAPQPPDVGSSDPLSMVGPSQGRSPSYAS

SEQ ID NO: 126 - DNA, 549 bp, Artificial Sequence
  FGF21 P78C
  CDS (1)..(549)
atgcatccaattccagattcttctccattattacaattcgggggccaagtccggcagcggtacctctacacagatgatgcccagcagacagaagcccacctggagatcagggaggatgggacggtggggggcgctgctgaccagagccccgaaagtctcctgcagctgaaagccttgaagccgggagttattcaaatcttgggagtcaagacatccaggttcctgtgccagcggtgcgatggggccctgtatggatcgctccactttgaccctgaggcctgcagcttccgggagctgcttcttgaggacggatacaatgtttaccagtccgaagcccacggcctcccgctgcacctgccagggaacaagtccccacaccgggaccctgcaccccgaggaccagctcgcttcctgccactaccaggcctgccccccgcacccccggagccacccggaatcctggccccccagccccccgatgtgggctcctcggaccctctgagcatggtgggaccttcccagggccgaagccccagctacgcttcctaa

SEQ ID NO: 127 - protein, 182 aa, Artificial Sequence
  Synthetic Construct
MHPIPDSSPLLQFGGQVRQRYLYTDDAQQTEAHLEIREDGTVGGAADQSPESLLQLKALKPGVIQILGVKTSRFLCQRCDGALYGSLHFDPEACSFRELLLEDGYNVYQSEAHGLPLHLPGNKSPHRDPAPRGPARFLPLPGLPPAPPEPPGILAPQPPDVGSSDPLSMVGPSQGRSPSYAS

SEQ ID NO: 128 - DNA, 549 bp, Artificial Sequence
  FGF21 P78R
  CDS (1)..(549)
atgcatccaattccagattcttctccattattacaattcgggggccaagtccggcagcggtacctctacacagatgatgcccagcagacagaagcccacctggagatcagggaggatgggacggtggggggcgctgctgaccagagccccgaaagtctcctgcagctgaaagccttgaagccgggagttattcaaatcttgggagtcaagacatccaggttcctgtgccagcggcgtgatggggccctgtatggatcgctccactttgaccctgaggcctgcagcttccgggagctgcttcttgaggacggatacaatgtttaccagtccgaagcccacggcctcccgctgcacctgccagggaacaagtccccacaccgggaccctgcaccccgaggaccagctcgcttcctgccactaccaggcctgccccccgcacccccggagccacccggaatcctggccccccagccccccgatgtgggctcctcggaccctctgagcatggtgggaccttcccagggccgaagccccagctacgcttcctaa

SEQ ID NO: 129 - protein, 182 aa, Artificial Sequence
  Synthetic Construct
MHPIPDSSPLLQFGGQVRQRYLYTDDAQQTEAHLEIREDGTVGGAADQSPESLLQLKALKPGVIQILGVKTSRFLCQRRDGALYGSLHFDPEACSFRELLLEDGYNVYQSEAHGLPLHLPGNKSPHRDPAPRGPARFLPLPGLPPAPPEPPGILAPQPPDVGSSDPLSMVGPSQGRSPSYAS

SEQ ID NO: 130 - DNA, 549 bp, Artificial Sequence
  FGF21 L86T
  CDS (1)..(549)
atgcatccaattccagattcttctccattattacaattcgggggccaagtccggcagcggtacctctacacagatgatgcccagcagacagaagcccacctggagatcagggaggatgggacggtggggggcgctgctgaccagagccccgaaagtctcctgcagctgaaagccttgaagccgggagttattcaaatcttgggagtcaagacatccaggttcctgtgccagcggccagatggggccctgtatggatcgacccactttgaccctgaggcctgcagcttccgggagctgcttcttgaggacggatacaatgtttaccagtccgaagcccacggcctcccgctgcacctgccagggaacaagtccccacaccgggaccctgcaccccgaggaccagctcgcttcctgccactaccaggcctgccccccgcacccccggagccacccggaatcctggccccccagccccccgatgtgggctcctcggaccctctgagcatggtgggaccttcccagggccgaagccccagctacgcttcctaa

SEQ ID NO: 131 - protein, 182 aa, Artificial Sequence
  Synthetic Construct
MHPIPDSSPLLQFGGQVRQRYLYTDDAQQTEAHLEIREDGTVGGAADQSPESLLQLKALKPGVIQILGVKTSRFLCQRPDGALYGSTHFDPEACSFRELLLEDGYNVYQSEAHGLPLHLPGNKSPHRDPAPRGPARFLPLPGLPPAPPEPPGILAPQPPDVGSSDPLSMVGPSQGRSPSYAS

SEQ ID NO: 132 - DNA, 549 bp, Artificial Sequence
  FGF21 L86C
  CDS (1)..(549)
atgcatccaattccagattcttctccattattacaattcgggggccaagtccggcagcggtacctctacacagatgatgcccagcagacagaagcccacctggagatcagggaggatgggacggtggggggcgctgctgaccagagccccgaaagtctcctgcagctgaaagccttgaagccgggagttattcaaatcttgggagtcaagacatccaggttcctgtgccagcggccagatggggccctgtatggatcgtgccactttgaccctgaggcctgcagcttccgggagctgcttcttgaggacggatacaatgtttaccagtccgaagcccacggcctcccgctgcacctgccagggaacaagtccccacaccgggaccctgcaccccgaggaccagctcgcttcctgccactaccaggcctgccccccgcacccccggagccacccggaatcctggccccccagccccccgatgtgggctcctcggaccctctgagcatggtgggaccttcccagggccgaagccccagctacgcttcctaa

SEQ ID NO: 133 - protein, 182 aa, Artificial Sequence
  Synthetic Construct
MHPIPDSSPLLQFGGQVRQRYLYTDDAQQTEAHLEIREDGTVGGAADQSPESLLQLKALKPGVIQILGVKTSRFLCQRPDGALYGSCHFDPEACSFRELLLEDGYNVYQSEAHGLPLHLPGNKSPHRDPAPRGPARFLPLPGLPPAPPEPPGILAPQPPDVGSSDPLSMVGPSQGRSPSYAS

SEQ ID NO: 134 - DNA, 549 bp, Artificial Sequence
  FGF21 L98C
  CDS (1)..(549)
atgcatccaattccagattcttctccattattacaattcgggggccaagtccggcagcggtacctctacacagatgatgcccagcagacagaagcccacctggagatcagggaggatgggacggtggggggcgctgctgaccagagccccgaaagtctcctgcagctgaaagccttgaagccgggagttattcaaatcttgggagtcaagacatccaggttcctgtgccagcggccagatggggccctgtatggatcgctccactttgaccctgaggcctgcagcttccgggagtgccttcttgaggacggatacaatgtttaccagtccgaagcccacggcctcccgctgcacctgccagggaacaagtccccacaccgggaccctgcaccccgaggaccagctcgcttcctgccactaccaggcctgccccccgcacccccggagccacccggaatcctggccccccagccccccgatgtgggctcctcggaccctctgagcatggtgggaccttcccagggccgaagccccagctacgcttcctaa

SEQ ID NO: 135 - protein, 182 aa, Artificial Sequence
  Synthetic Construct
MHPIPDSSPLLQFGGQVRQRYLYTDDAQQTEAHLEIREDGTVGGAADQSPESLLQLKALKPGVIQILGVKTSRFLCQRPDGALYGSLHFDPEACSFRECLLEDGYNVYQSEAHGLPLHLPGNKSPHRDPAPRGPARFLPLPGLPPAPPEPPGILAPQPPDVGSSDPLSMVGPSQGRSPSYAS

SEQ ID NO: 136 - DNA, 549 bp, Artificial Sequence
  FGF21 L98R
  CDS (1)..(549)
atgcatccaattccagattcttctccattattacaattcgggggccaagtccggcagcggtacctctacacagatgatgcccagcagacagaagcccacctggagatcagggaggatgggacggtggggggcgctgctgaccagagccccgaaagtctcctgcagctgaaagccttgaagccgggagttattcaaatcttgggagtcaagacatccaggttcctgtgccagcggccagatggggccctgtatggatcgctccactttgaccctgaggcctgcagcttccgggagcgtcttcttgaggacggatacaatgtttaccagtccgaagcccacggcctcccgctgcacctgccagggaacaagtccccacaccgggaccctgcaccccgaggaccagctcgcttcctgccactaccaggcctgccccccgcacccccggagccacccggaatcctggccccccagccccccgatgtgggctcctcggaccctctgagcatggtgggaccttcccagggccgaagccccagctacgcttcctaa

SEQ ID NO: 137 - protein, 182 aa, Artificial Sequence
  Synthetic Construct
MHPIPDSSPLLQFGGQVRQRYLYTDDAQQTEAHLEIREDGTVGGAADQSPESLLQLKALKPGVIQILGVKTSRFLCQRPDGALYGSLHFDPEACSFRERLLEDGYNVYQSEAHGLPLHLPGNKSPHRDPAPRGPARFLPLPGLPPAPPEPPGILAPQPPDVGSSDPLSMVGPSQGRSPSYAS

SEQ ID NO: 138 - DNA, 549 bp, Artificial Sequence
  FGF21 L52T
  CDS (1)..(549)
atgcatccaattccagattcttctccattattacaattcgggggccaagtccggcagcggtacctctacacagatgatgcccagcagacagaagcccacctggagatcagggaggatgggacggtggggggcgctgctgaccagagccccgaaagtaccctgcagctgaaagccttgaagccgggagttattcaaatcttgggagtcaagacatccaggttcctgtgccagcggccagatggggccctgtatggatcgctccactttgaccctgaggcctgcagcttccgggagctgcttcttgaggacggatacaatgtttaccagtccgaagcccacggcctcccgctgcacctgccagggaacaagtccccacaccgggaccctgcaccccgaggaccagctcgcttcctgccactaccaggcctgccccccgcacccccggagccacccggaatcctggccccccagccccccgatgtgggctcctcggaccctctgagcatggtgggaccttcccagggccgaagccccagctacgcttcctaa

SEQ ID NO: 139 - protein, 182 aa, Artificial Sequence
  Synthetic Construct
MHPIPDSSPLLQFGGQVRQRYLYTDDAQQTEAHLEIREDGTVGGAADQSPESTLQLKALKPGVIQILGVKTSRFLCQRPDGALYGSLHFDPEACSFRELLLEDGYNVYQSEAHGLPLHLPGNKSPHRDPAPRGPARFLPLPGLPPAPPEPPGILAPQPPDVGSSDPLSMVGPSQGRSPSYAS

SEQ ID NO: 140 - DNA, 549 bp, Artificial Sequence
  FGF21 L58E
  CDS (1)..(549)
atgcatccaattccagattcttctccattattacaattcgggggccaagtccggcagcggtacctctacacagatgatgcccagcagacagaagcccacctggagatcagggaggatgggacggtggggggcgctgctgaccagagccccgaaagtctcctgcagctgaaagccgaaaagccgggagttattcaaatcttgggagtcaagacatccaggttcctgtgccagcggccagatggggccctgtatggatcgctccactttgaccctgaggcctgcagcttccgggagctgcttcttgaggacggatacaatgtttaccagtccgaagcccacggcctcccgctgcacctgccagggaacaagtccccacaccgggaccctgcaccccgaggaccagctcgcttcctgccactaccaggcctgccccccgcacccccggagccacccggaatcctggccccccagccccccgatgtgggctcctcggaccctctgagcatggtgggaccttcccagggccgaagccccagctacgcttcctaa

SEQ ID NO: 141 - protein, 182 aa, Artificial Sequence
  Synthetic Construct
MHPIPDSSPLLQFGGQVRQRYLYTDDAQQTEAHLEIREDGTVGGAADQSPESLLQLKAEKPGVIQILGVKTSRFLCQRPDGALYGSLHFDPEACSFRELLLEDGYNVYQSEAHGLPLHLPGNKSPHRDPAPRGPARFLPLPGLPPAPPEPPGILAPQPPDVGSSDPLSMVGPSQGRSPSYAS

SEQ ID NO: 142 - DNA, 1278 bp, Artificial Sequence
  Fc-L15-L98R P171G 182P
  CDS (1)..(1278)
atggacaaaactcacacatgtccaccttgtccagctccggaactcctggggggaccgtcagtcttcctcttccccccaaaacccaaggacaccctcatgatctcccgtacccctgaggtcacatgcgtggtggtggacgtgagccacgaagaccctgaggtcaagttcaactggtacgtggacggcgtggaggtgcataatgccaagacaaagccgcgtgaggagcagtacaacagcacgtaccgtgtggtcagcgtcctcaccgtcctgcaccaggactggctgaatggcaaggagtacaagtgcaaggtctccaacaaagccctcccagcccccatcgagaaaaccatctccaaagccaaagggcagccccgagaaccacaggtgtacaccctgcccccatcccgtgatgagctgaccaagaaccaggtcagcctgacctgcctggtcaaaggcttctatcccagcgacatcgccgtggagtgggagagcaatgggcagccggagaacaactacaagaccacgcctcccgtgctggactccgacggctccttcttcctctacagcaagctcaccgtggacaagagccgttggcagcaggggaacgtcttctcatgctccgtgatgcatgaggctctgcacaaccactacacgcagaagagcctctccctgtctccgggtaaaggtggaggtggtggttctggtggtggtagcggtggtggtggatcccatccaattccagattcttctccattattacaattcgggggccaagtccggcagcggtacctctacacagatgatgcccagcagacagaagcccacctggagatcagggaggatgggacggtggggggcgctgctgaccagagccccgaaagtctcctgcagctgaaagccttgaagccgggagttattcaaatcttgggagtcaagacatccaggttcctgtgccagcggccagatggggccctgtatggatcgctccactttgaccctgaggcctgcagcttccgggagcgtcttcttgaggacggatacaatgtttaccagtccgaagcccacggcctcccgctgcacctgccagggaacaagtccccacaccgggaccctgcaccccgaggaccagctcgcttcctgccactaccaggcctgccccccgcacccccggagccacccggaatcctggccccccagccccccgatgtgggctcctcggaccctctgagcatggtgggaggttcccagggccgaagccccagctacgcttccccgtaa

SEQ ID NO: 143 - protein, 425 aa, Artificial Sequence
  Synthetic Construct
MDKTHTCPPCPAPELLGGPSVFLFPPKPKDTLMISRTPEVTCVVVDVSHEDPEVKFNWYVDGVEVHNAKTKPREEQYNSTYRVVSVLTVLHQDWLNGKEYKCKVSNKALPAPIEKTISKAKGQPREPQVYTLPPSRDELTKNQVSLTCLVKGFYPSDIAVEWESNGQPENNYKTTPPVLDSDGSFFLYSKLTVDKSRWQQGNVFSCSVMHEALHNHYTQKSLSLSPGKGGGGGSGGGSGGGGSHPIPDSSPLLQFGGQVRQRYLYTDDAQQTEAHLEIREDGTVGGAADQSPESLLQLKALKPGVIQILGVKTSRFLCQRPDGALYGSLHFDPEACSFRERLLEDGYNVYQSEAHGLPLHLPGNKSPHRDPAPRGPARFLPLPGLPPAPPEPPGILAPQPPDVGSSDPLSMVGGSQGRSPSYASP

SEQ ID NO: 144 - DNA, 1278 bp, Artificial Sequence
  Fc-L15-L98R P171G 182G
  CDS (1)..(1278)
atggacaaaactcacacatgtccaccttgtccagctccggaactcctggggggaccgtcagtcttcctcttccccccaaaacccaaggacaccctcatgatctcccgtacccctgaggtcacatgcgtggtggtggacgtgagccacgaagaccctgaggtcaagttcaactggtacgtggacggcgtggaggtgcataatgccaagacaaagccgcgtgaggagcagtacaacagcacgtaccgtgtggtcagcgtcctcaccgtcctgcaccaggactggctgaatggcaaggagtacaagtgcaaggtctccaacaaagccctcccagcccccatcgagaaaaccatctccaaagccaaagggcagccccgagaaccacaggtgtacaccctgcccccatcccgtgatgagctgaccaagaaccaggtcagcctgacctgcctggtcaaaggcttctatcccagcgacatcgccgtggagtgggagagcaatgggcagccggagaacaactacaagaccacgcctcccgtgctggactccgacggctccttcttcctctacagcaagctcaccgtggacaagagccgttggcagcaggggaacgtcttctcatgctccgtgatgcatgaggctctgcacaaccactacacgcagaagagcctctccctgtctccgggtaaaggtggaggtggtggttctggtggtggtagcggtggtggtggatcccatccaattccagattcttctccattattacaattcgggggccaagtccggcagcggtacctctacacagatgatgcccagcagacagaagcccacctggagatcagggaggatgggacggtggggggcgctgctgaccagagccccgaaagtctcctgcagctgaaagccttgaagccgggagttattcaaatcttgggagtcaagacatccaggttcctgtgccagcggccagatggggccctgtatggatcgctccactttgaccctgaggcctgcagcttccgggagcgtcttcttgaggacggatacaatgtttaccagtccgaagcccacggcctcccgctgcacctgccagggaacaagtccccacaccgggaccctgcaccccgaggaccagctcgcttcctgccactaccaggcctgccccccgcacccccggagccacccggaatcctggccccccagccccccgatgtgggctcctcggaccctctgagcatggtgggaggttcccagggccgaagccccagctacgcttccggctaa

SEQ ID NO: 145 - protein, 425 aa, Artificial Sequence
  Synthetic Construct
MDKTHTCPPCPAPELLGGPSVFLFPPKPKDTLMISRTPEVTCVVVDVSHEDPEVKFNWYVDGVEVHNAKTKPREEQYNSTYRVVSVLTVLHQDWLNGKEYKCKVSNKALPAPIEKTISKAKGQPREPQVYTLPPSRDELTKNQVSLTCLVKGFYPSDIAVEWESNGQPENNYKTTPPVLDSDGSFFLYSKLTVDKSRWQQGNVFSCSVMHEALHNHYTQKSLSLSPGKGGGGGSGGGSGGGGSHPIPDSSPLLQFGGQVRQRYLYTDDAQQTEAHLEIREDGTVGGAADQSPESLLQLKALKPGVIQILGVKTSRFLCQRPDGALYGSLHFDPEACSFRERLLEDGYNVYQSEAHGLPLHLPGNKSPHRDPAPRGPARFLPLPGLPPAPPEPPGILAPQPPDVGSSDPLSMVGGSQGRSPSYASG

SEQ ID NO: 146 - DNA, 1281 bp, Artificial Sequence
  Fc-L15-L98R P171G 182G 183G
  CDS (1)..(1281)
atggacaaaactcacacatgtccaccttgtccagctccggaactcctggggggaccgtcagtcttcctcttccccccaaaacccaaggacaccctcatgatctcccgtacccctgaggtcacatgcgtggtggtggacgtgagccacgaagaccctgaggtcaagttcaactggtacgtggacggcgtggaggtgcataatgccaagacaaagccgcgtgaggagcagtacaacagcacgtaccgtgtggtcagcgtcctcaccgtcctgcaccaggactggctgaatggcaaggagtacaagtgcaaggtctccaacaaagccctcccagcccccatcgagaaaaccatctccaaagccaaagggcagccccgagaaccacaggtgtacaccctgcccccatcccgtgatgagctgaccaagaaccaggtcagcctgacctgcctggtcaaaggcttctatcccagcgacatcgccgtggagtgggagagcaatgggcagccggagaacaactacaagaccacgcctcccgtgctggactccgacggctccttcttcctctacagcaagctcaccgtggacaagagccgttggcagcaggggaacgtcttctcatgctccgtgatgcatgaggctctgcacaaccactacacgcagaagagcctctccctgtctccgggtaaaggtggaggtggtggttctggtggtggtagcggtggtggtggatcccatccaattccagattcttctccattattacaattcgggggccaagtccggcagcggtacctctacacagatgatgcccagcagacagaagcccacctggagatcagggaggatgggacggtggggggcgctgctgaccagagccccgaaagtctcctgcagctgaaagccttgaagccgggagttattcaaatcttgggagtcaagacatccaggttcctgtgccagcggccagatggggccctgtatggatcgctccactttgaccctgaggcctgcagcttccgggagcgtcttcttgaggacggatacaatgtttaccagtccgaagcccacggcctcccgctgcacctgccagggaacaagtccccacaccgggaccctgcaccccgaggaccagctcgcttcctgccactaccaggcctgccccccgcacccccggagccacccggaatcctggccccccagccccccgatgtgggctcctcggaccctctgagcatggtgggaggttcccagggccgaagccccagctacgcttccggtggctaa

SEQ ID NO: 147 - protein, 426 aa, Artificial Sequence
  Synthetic Construct
MDKTHTCPPCPAPELLGGPSVFLFPPKPKDTLMISRTPEVTCVVVDVSHEDPEVKFNWYVDGVEVHNAKTKPREEQYNSTYRVVSVLTVLHQDWLNGKEYKCKVSNKALPAPIEKTISKAKGQPREPQVYTLPPSRDELTKNQVSLTCLVKGFYPSDIAVEWESNGQPENNYKTTPPVLDSDGSFFLYSKLTVDKSRWQQGNVFSCSVMHEALHNHYTQKSLSLSPGKGGGGGSGGGSGGGGSHPIPDSSPLLQFGGQVRQRYLYTDDAQQTEAHLEIREDGTVGGAADQSPESLLQLKALKPGVIQILGVKTSRFLCQRPDGALYGSLHFDPEACSFRERLLEDGYNVYQSEAHGLPLHLPGNKSPHRDPAPRGPARFLPLPGLPPAPPEPPGILAPQPPDVGSSDPLSMVGGSQGRSPSYASGG

SEQ ID NO: 148 - DNA, 1275 bp, Artificial Sequence
  Fc-L15-L98R P171G Y179S
  CDS (1)..(1275)
atggacaaaactcacacatgtccaccttgtccagctccggaactcctggggggaccgtcagtcttcctcttccccccaaaacccaaggacaccctcatgatctcccgtacccctgaggtcacatgcgtggtggtggacgtgagccacgaagaccctgaggtcaagttcaactggtacgtggacggcgtggaggtgcataatgccaagacaaagccgcgtgaggagcagtacaacagcacgtaccgtgtggtcagcgtcctcaccgtcctgcaccaggactggctgaatggcaaggagtacaagtgcaaggtctccaacaaagccctcccagcccccatcgagaaaaccatctccaaagccaaagggcagccccgagaaccacaggtgtacaccctgcccccatcccgtgatgagctgaccaagaaccaggtcagcctgacctgcctggtcaaaggcttctatcccagcgacatcgccgtggagtgggagagcaatgggcagccggagaacaactacaagaccacgcctcccgtgctggactccgacggctccttcttcctctacagcaagctcaccgtggacaagagccgttggcagcaggggaacgtcttctcatgctccgtgatgcatgaggctctgcacaaccactacacgcagaagagcctctccctgtctccgggtaaaggtggaggtggtggttctggtggtggtagcggtggtggtggatcccatccaattccagattcttctccattattacaattcgggggccaagtccggcagcggtacctctacacagatgatgcccagcagacagaagcccacctggagatcagggaggatgggacggtggggggcgctgctgaccagagccccgaaagtctcctgcagctgaaagccttgaagccgggagttattcaaatcttgggagtcaagacatccaggttcctgtgccagcggccagatggggccctgtatggatcgctccactttgaccctgaggcctgcagcttccgggagcgtcttcttgaggacggatacaatgtttaccagtccgaagcccacggcctcccgctgcacctgccagggaacaagtccccacaccgggaccctgcaccccgaggaccagctcgcttcctgccactaccaggcctgccccccgcacccccggagccacccggaatcctggccccccagccccccgatgtgggctcctcggaccctctgagcatggtgggaggttcccagggccgaagccccagctccgcttcctaa

SEQ ID NO: 149 - protein, 424 aa, Artificial Sequence
  Synthetic Construct
MDKTHTCPPCPAPELLGGPSVFLFPPKPKDTLMISRTPEVTCVVVDVSHEDPEVKFNWYVDGVEVHNAKTKPREEQYNSTYRVVSVLTVLHQDWLNGKEYKCKVSNKALPAPIEKTISKAKGQPREPQVYTLPPSRDELTKNQVSLTCLVKGFYPSDIAVEWESNGQPENNYKTTPPVLDSDGSFFLYSKLTVDKSRWQQGNVFSCSVMHEALHNHYTQKSLSLSPGKGGGGGSGGGSGGGGSHPIPDSSPLLQFGGQVRQRYLYTDDAQQTEAHLEIREDGTVGGAADQSPESLLQLKALKPGVIQILGVKTSRFLCQRPDGALYGSLHFDPEACSFRERLLEDGYNVYQSEAHGLPLHLPGNKSPHRDPAPRGPARFLPLPGLPPAPPEPPGILAPQPPDVGSSDPLSMVGGSQGRSPSSAS

SEQ ID NO: 150 - DNA, 1275 bp, Artificial Sequence
  Fc-L15-L98R P171G Y179F
  CDS (1)..(1275)
atggacaaaactcacacatgtccaccttgtccagctccggaactcctggggggaccgtcagtcttcctcttccccccaaaacccaaggacaccctcatgatctcccgtacccctgaggtcacatgcgtggtggtggacgtgagccacgaagaccctgaggtcaagttcaactggtacgtggacggcgtggaggtgcataatgccaagacaaagccgcgtgaggagcagtacaacagcacgtaccgtgtggtcagcgtcctcaccgtcctgcaccaggactggctgaatggcaaggagtacaagtgcaaggtctccaacaaagccctcccagcccccatcgagaaaaccatctccaaagccaaagggcagccccgagaaccacaggtgtacaccctgcccccatcccgtgatgagctgaccaagaaccaggtcagcctgacctgcctggtcaaaggcttctatcccagcgacatcgccgtggagtgggagagcaatgggcagccggagaacaactacaagaccacgcctcccgtgctggactccgacggctccttcttcctctacagcaagctcaccgtggacaagagccgttggcagcaggggaacgtcttctcatgctccgtgatgcatgaggctctgcacaaccactacacgcagaagagcctctccctgtctccgggtaaaggtggaggtggtggttctggtggtggtagcggtggtggtggatcccatccaattccagattcttctccattattacaattcgggggccaagtccggcagcggtacctctacacagatgatgcccagcagacagaagcccacctggagatcagggaggatgggacggtggggggcgctgctgaccagagccccgaaagtctcctgcagctgaaagccttgaagccgggagttattcaaatcttgggagtcaagacatccaggttcctgtgccagcggccagatggggccctgtatggatcgctccactttgaccctgaggcctgcagcttccgggagcgtcttcttgaggacggatacaatgtttaccagtccgaagcccacggcctcccgctgcacctgccagggaacaagtccccacaccgggaccctgcaccccgaggaccagctcgcttcctgccactaccaggcctgccccccgcacccccggagccacccggaatcctggccccccagccccccgatgtgggctcctcggaccctctgagcatggtgggaggttcccagggccgaagccccagcttcgcttcctaa

SEQ ID NO: 151 - protein, 424 aa, Artificial Sequence
  Synthetic Construct
MDKTHTCPPCPAPELLGGPSVFLFPPKPKDTLMISRTPEVTCVVVDVSHEDPEVKFNWYVDGVEVHNAKTKPREEQYNSTYRVVSVLTVLHQDWLNGKEYKCKVSNKALPAPIEKTISKAKGQPREPQVYTLPPSRDELTKNQVSLTCLVKGFYPSDIAVEWESNGQPENNYKTTPPVLDSDGSFFLYSKLTVDKSRWQQGNVFSCSVMHEALHNHYTQKSLSLSPGKGGGGGSGGGSGGGGSHPIPDSSPLLQFGGQVRQRYLYTDDAQQTEAHLEIREDGTVGGAADQSPESLLQLKALKPGVIQILGVKTSRFLCQRPDGALYGSLHFDPEACSFRERLLEDGYNVYQSEAHGLPLHLPGNKSPHRDPAPRGPARFLPLPGLPPAPPEPPGILAPQPPDVGSSDPLSMVGGSQGRSPSFAS

SEQ ID NO: 152 - DNA, 1275 bp, Artificial Sequence
  Fc-L15-L98R P171G Y179A
  CDS (1)..(1275)
atggacaaaactcacacatgtccaccttgtccagctccggaactcctggggggaccgtcagtcttcctcttccccccaaaacccaaggacaccctcatgatctcccgtacccctgaggtcacatgcgtggtggtggacgtgagccacgaagaccctgaggtcaagttcaactggtacgtggacggcgtggaggtgcataatgccaagacaaagccgcgtgaggagcagtacaacagcacgtaccgtgtggtcagcgtcctcaccgtcctgcaccaggactggctgaatggcaaggagtacaagtgcaaggtctccaacaaagccctcccagcccccatcgagaaaaccatctccaaagccaaagggcagccccgagaaccacaggtgtacaccctgcccccatcccgtgatgagctgaccaagaaccaggtcagcctgacctgcctggtcaaaggcttctatcccagcgacatcgccgtggagtgggagagcaatgggcagccggagaacaactacaagaccacgcctcccgtgctggactccgacggctccttcttcctctacagcaagctcaccgtggacaagagccgttggcagcaggggaacgtcttctcatgctccgtgatgcatgaggctctgcacaaccactacacgcagaagagcctctccctgtctccgggtaaaggtggaggtggtggttctggtggtggtagcggtggtggtggatcccatccaattccagattcttctccattattacaattcgggggccaagtccggcagcggtacctctacacagatgatgcccagcagacagaagcccacctggagatcagggaggatgggacggtggggggcgctgctgaccagagccccgaaagtctcctgcagctgaaagccttgaagccgggagttattcaaatcttgggagtcaagacatccaggttcctgtgccagcggccagatggggccctgtatggatcgctccactttgaccctgaggcctgcagcttccgggagcgtcttcttgaggacggatacaatgtttaccagtccgaagcccacggcctcccgctgcacctgccagggaacaagtccccacaccgggaccctgcaccccgaggaccagctcgcttcctgccactaccaggcctgccccccgcacccccggagccacccggaatcctggccccccagccccccgatgtgggctcctcggaccctctgagcatggtgggaggttcccagggccgaagccccagcgctgcttcctaa

SEQ ID NO: 153 - protein, 424 aa, Artificial Sequence
  Synthetic Construct
MDKTHTCPPCPAPELLGGPSVFLFPPKPKDTLMISRTPEVTCVVVDVSHEDPEVKFNWYVDGVEVHNAKTKPREEQYNSTYRVVSVLTVLHQDWLNGKEYKCKVSNKALPAPIEKTISKAKGQPREPQVYTLPPSRDELTKNQVSLTCLVKGFYPSDIAVEWESNGQPENNYKTTPPVLDSDGSFFLYSKLTVDKSRWQQGNVFSCSVMHEALHNHYTQKSLSLSPGKGGGGGSGGGSGGGGSHPIPDSSPLLQFGGQVRQRYLYTDDAQQTEAHLEIREDGTVGGAADQSPESLLQLKALKPGVIQILGVKTSRFLCQRPDGALYGSLHFDPEACSFRERLLEDGYNVYQSEAHGLPLHLPGNKSPHRDPAPRGPARFLPLPGLPPAPPEPPGILAPQPPDVGSSDPLSMVGGSQGRSPSAAS

SEQ ID NO: 154 - DNA, 1275 bp, Artificial Sequence
  Fc-L15-L98R P171G A180S
  CDS (1)..(1275)
atggacaaaactcacacatgtccaccttgtccagctccggaactcctggggggaccgtcagtcttcctcttccccccaaaacccaaggacaccctcatgatctcccgtacccctgaggtcacatgcgtggtggtggacgtgagccacgaagaccctgaggtcaagttcaactggtacgtggacggcgtggaggtgcataatgccaagacaaagccgcgtgaggagcagtacaacagcacgtaccgtgtggtcagcgtcctcaccgtcctgcaccaggactggctgaatggcaaggagtacaagtgcaaggtctccaacaaagccctcccagcccccatcgagaaaaccatctccaaagccaaagggcagccccgagaaccacaggtgtacaccctgcccccatcccgtgatgagctgaccaagaaccaggtcagcctgacctgcctggtcaaaggcttctatcccagcgacatcgccgtggagtgggagagcaatgggcagccggagaacaactacaagaccacgcctcccgtgctggactccgacggctccttcttcctctacagcaagctcaccgtggacaagagccgttggcagcaggggaacgtcttctcatgctccgtgatgcatgaggctctgcacaaccactacacgcagaagagcctctccctgtctccgggtaaaggtggaggtggtggttctggtggtggtagcggtggtggtggatcccatccaattccagattcttctccattattacaattcgggggccaagtccggcagcggtacctctacacagatgatgcccagcagacagaagcccacctggagatcagggaggatgggacggtggggggcgctgctgaccagagccccgaaagtctcctgcagctgaaagccttgaagccgggagttattcaaatcttgggagtcaagacatccaggttcctgtgccagcggccagatggggccctgtatggatcgctccactttgaccctgaggcctgcagcttccgggagcgtcttcttgaggacggatacaatgtttaccagtccgaagcccacggcctcccgctgcacctgccagggaacaagtccccacaccgggaccctgcaccccgaggaccagctcgcttcctgccactaccaggcctgccccccgcacccccggagccacccggaatcctggccccccagccccccgatgtgggctcctcggaccctctgagcatggtgggaggttcccagggccgaagccccagctactcctcctaa

SEQ ID NO: 155 - protein, 424 aa, Artificial Sequence
  Synthetic Construct
MDKTHTCPPCPAPELLGGPSVFLFPPKPKDTLMISRTPEVTCVVVDVSHEDPEVKFNWYVDGVEVHNAKTKPREEQYNSTYRVVSVLTVLHQDWLNGKEYKCKVSNKALPAPIEKTISKAKGQPREPQVYTLPPSRDELTKNQVSLTCLVKGFYPSDIAVEWESNGQPENNYKTTPPVLDSDGSFFLYSKLTVDKSRWQQGNVFSCSVMHEALHNHYTQKSLSLSPGKGGGGGSGGGSGGGGSHPIPDSSPLLQFGGQVRQRYLYTDDAQQTEAHLEIREDGTVGGAADQSPESLLQLKALKPGVIQILGVKTSRFLCQRPDGALYGSLHFDPEACSFRERLLEDGYNVYQSEAHGLPLHLPGNKSPHRDPAPRGPARFLPLPGLPPAPPEPPGILAPQPPDVGSSDPLSMVGGSQGRSPSYSS

SEQ ID NO: 156 - DNA, 1275 bp, Artificial Sequence
  Fc-L15-L98R P171G A180G
  CDS (1)..(1275)
atggacaaaactcacacatgtccaccttgtccagctccggaactcctggggggaccgtcagtcttcctcttccccccaaaacccaaggacaccctcatgatctcccgtacccctgaggtcacatgcgtggtggtggacgtgagccacgaagaccctgaggtcaagttcaactggtacgtggacggcgtggaggtgcataatgccaagacaaagccgcgtgaggagcagtacaacagcacgtaccgtgtggtcagcgtcctcaccgtcctgcaccaggactggctgaatggcaaggagtacaagtgcaaggtctccaacaaagccctcccagcccccatcgagaaaaccatctccaaagccaaagggcagccccgagaaccacaggtgtacaccctgcccccatcccgtgatgagctgaccaagaaccaggtcagcctgacctgcctggtcaaaggcttctatcccagcgacatcgccgtggagtgggagagcaatgggcagccggagaacaactacaagaccacgcctcccgtgctggactccgacggctccttcttcctctacagcaagctcaccgtggacaagagccgttggcagcaggggaacgtcttctcatgctccgtgatgcatgaggctctgcacaaccactacacgcagaagagcctctccctgtctccgggtaaaggtggaggtggtggttctggtggtggtagcggtggtggtggatcccatccaattccagattcttctccattattacaattcgggggccaagtccggcagcggtacctctacacagatgatgcccagcagacagaagcccacctggagatcagggaggatgggacggtggggggcgctgctgaccagagccccgaaagtctcctgcagctgaaagccttgaagccgggagttattcaaatcttgggagtcaagacatccaggttcctgtgccagcggccagatggggccctgtatggatcgctccactttgaccctgaggcctgcagcttccgggagcgtcttcttgaggacggatacaatgtttaccagtccgaagcccacggcctcccgctgcacctgccagggaacaagtccccacaccgggaccctgcaccccgaggaccagctcgcttcctgccactaccaggcctgccccccgcacccccggagccacccggaatcctggccccccagccccccgatgtgggctcctcggaccctctgagcatggtgggaggttcccagggccgaagccccagctacggttcctaa

SEQ ID NO: 157 - protein, 424 aa, Artificial Sequence
  Synthetic Construct
MDKTHTCPPCPAPELLGGPSVFLFPPKPKDTLMISRTPEVTCVVVDVSHEDPEVKFNWYVDGVEVHNAKTKPREEQYNSTYRVVSVLTVLHQDWLNGKEYKCKVSNKALPAPIEKTISKAKGQPREPQVYTLPPSRDELTKNQVSLTCLVKGFYPSDIAVEWESNGQPENNYKTTPPVLDSDGSFFLYSKLTVDKSRWQQGNVFSCSVMHEALHNHYTQKSLSLSPGKGGGGGSGGGSGGGGSHPIPDSSPLLQFGGQVRQRYLYTDDAQQTEAHLEIREDGTVGGAADQSPESLLQLKALKPGVIQILGVKTSRFLCQRPDGALYGSLHFDPEACSFRERLLEDGYNVYQSEAHGLPLHLPGNKSPHRDPAPRGPARFLPLPGLPPAPPEPPGILAPQPPDVGSSDPLSMVGGSQGRSPSYGS

SEQ ID NO: 158 - DNA, 1287 bp, Artificial Sequence
  MKEDD-FGF21-(L15)-Fc
  CDS (1)..(1287)
atgaaagaagatgatcacccaattccagattcttctccattattacaattcgggggccaagtccggcagcggtacctctacacagatgatgcccagcagacagaagcccacctggagatcagggaggatgggacggtggggggcgctgctgaccagagccccgaaagtctcctgcagctgaaagccttgaagccgggagttattcaaatcttgggagtcaagacatccaggttcctgtgccagcggccagatggggccctgtatggatcgctccactttgaccctgaggcctgcagcttccgggagctgcttcttgaggacggatacaatgtttaccagtccgaagcccacggcctcccgctgcacctgccagggaacaagtccccacaccgggaccctgcaccccgaggaccagctcgcttcctgccactaccaggcctgccacccgcacccccggagccacccggaatcctggccccccagccccccgatgtgggctcctcggaccctctgagcatggtgggaccttcccagggccgaagccccagctacgcttccggtggaggtggtggttctggtggtggtagcggtggtggtggatccgacaaaactcacacatgcccaccgtgcccagcacctgaactcctggggggaccgtcagtcttcctcttccccccaaaacccaaggacaccctcatgatctcccgtacccctgaggtcacatgcgtggtggtggacgtgagccacgaagaccctgaggtcaagttcaactggtacgtggacggcgtggaggtgcataatgccaagacaaagccgcgtgaggagcagtacaacagcacgtaccgtgtggtcagcgtcctcaccgtcctgcaccaggactggctgaatggcaaggagtacaagtgcaaggtctccaacaaagccctcccagcccccatcgagaaaaccatctccaaagccaaagggcagccccgagaaccacaggtgtacaccctgcccccatcccgggatgagctgaccaagaaccaggtcagcctgacctgcctggtcaaaggcttctatcccagcgacatcgccgtggagtgggagagcaatgggcagccggagaacaactacaagaccacgcctcccgtgctggactccgacggctccttcttcctctatagcaagctcaccgtggacaagagcaggtggcagcaggggaacgtcttctcatgctccgtgatgcatgaggctctgcacaaccactacacgcagaagagcctctccctgtctccgggtaaataa

SEQ ID NO: 159 - protein, 428 aa, Artificial Sequence
  Synthetic Construct
MKEDDHPIPDSSPLLQFGGQVRQRYLYTDDAQQTEAHLEIREDGTVGGAADQSPESLLQLKALKPGVIQILGVKTSRFLCQRPDGALYGSLHFDPEACSFRELLLEDGYNVYQSEAHGLPLHLPGNKSPHRDPAPRGPARFLPLPGLPPAPPEPPGILAPQPPDVGSSDPLSMVGPSQGRSPSYASGGGGGSGGGSGGGGSDKTHTCPPCPAPELLGGPSVFLFPPKPKDTLMISRTPEVTCVVVDVSHEDPEVKFNWYVDGVEVHNAKTKPREEQYNSTYRVVSVLTVLHQDWLNGKEYKCKVSNKALPAPIEKTISKAKGQPREPQVYTLPPSRDELTKNQVSLTCLVKGFYPSDIAVEWESNGQPENNYKTTPPVLDSDGSFFLYSKLTVDKSRWQQGNVFSCSVMHEALHNHYTQKSLSLSPGK

SEQ ID NO: 160 - DNA, 630 bp, Artificial Sequence
  FGF21 Y179N S181T, 28AA signal sequence removed during processing
  CDS (1)..(630)
atggactcggacgagaccgggttcgagcactcaggactgtgggtttctgtgctggctggtcttctgctgggagcctgccaggcacaccccatccctgactccagtcctctcctgcaattcgggggccaagtccggcagcggtacctctacacagatgatgcccagcagacagaagcccacctggagatcagggaggatgggacggtggggggcgctgctgaccagagccccgaaagtctcctgcagctgaaagccttgaagccgggagttattcaaatcttgggagtcaagacatccaggttcctgtgccagcggccagatggggccctgtatggatcgctccactttgaccctgaggcctgcagcttccgggagctgcttcttgaggacggatacaatgtttaccagtccgaagcccacggcctcccgctgcacctgccagggaacaagtccccacaccgggaccctgcaccccgaggaccagctcgcttcctgccactaccaggcctgccacccgcacccccggagccacccggaatcctggccccccagccccccgatgtgggctcctcggaccctctgagcatggtgggaccttcccagggccgaagccccagcaacgctacctga

SEQ ID NO: 161 - protein, 209 aa, Artificial Sequence
  Synthetic Construct
MDSDETGFEHSGLWVSVLAGLLLGACQAHPIPDSSPLLQFGGQVRQRYLYTDDAQQTEAHLEIREDGTVGGAADQSPESLLQLKALKPGVIQILGVKTSRFLCQRPDGALYGSLHFDPEACSFRELLLEDGYNVYQSEAHGLPLHLPGNKSPHRDPAPRGPARFLPLPGLPPAPPEPPGILAPQPPDVGSSDPLSMVGPSQGRSPSNAT

SEQ ID NO: 162 - DNA, 630 bp, Artificial Sequence
  FGF21 Y179N, 28 AA signal sequence removed during processing
  CDS (1)..(630)
atggactcggacgagaccgggttcgagcactcaggactgtgggtttctgtgctggctggtcttctgctgggagcctgccaggcacaccccatccctgactccagtcctctcctgcaattcgggggccaagtccggcagcggtacctctacacagatgatgcccagcagacagaagcccacctggagatcagggaggatgggacggtggggggcgctgctgaccagagccccgaaagtctcctgcagctgaaagccttgaagccgggagttattcaaatcttgggagtcaagacatccaggttcctgtgccagcggccagatggggccctgtatggatcgctccactttgaccctgaggcctgcagcttccgggagctgcttcttgaggacggatacaatgtttaccagtccgaagcccacggcctcccgctgcacctgccagggaacaagtccccacaccgggaccctgcaccccgaggaccagctcgcttcctgccactaccaggcctgccacccgcacccccggagccacccggaatcctggccccccagccccccgatgtgggctcctcggaccctctgagcatggtgggaccttcccagggccgaagccccagcaacgcttcctga

SEQ ID NO: 163 - protein, 209 aa, Artificial Sequence
  Synthetic Construct
MDSDETGFEHSGLWVSVLAGLLLGACQAHPIPDSSPLLQFGGQVRQRYLYTDDAQQTEAHLEIREDGTVGGAADQSPESLLQLKALKPGVIQILGVKTSRFLCQRPDGALYGSLHFDPEACSFRELLLEDGYNVYQSEAHGLPLHLPGNKSPHRDPAPRGPARFLPLPGLPPAPPEPPGILAPQPPDVGSSDPLSMVGPSQGRSPSNAS

SEQ ID NO: 164 - DNA, 630 bp, Artificial Sequence
  FGF21 P124S, 28 AA signal sequence removed during processing
  CDS (1)..(630)
atggactcggacgagaccgggttcgagcactcaggactgtgggtttctgtgctggctggtcttctgctgggagcctgccaggcacaccccatccctgactccagtcctctcctgcaattcgggggccaagtccggcagcggtacctctacacagatgatgcccagcagacagaagcccacctggagatcagggaggatgggacggtggggggcgctgctgaccagagccccgaaagtctcctgcagctgaaagccttgaagccgggagttattcaaatcttgggagtcaagacatccaggttcctgtgccagcggccagatggggccctgtatggatcgctccactttgaccctgaggcctgcagcttccgggagctgcttcttgaggacggatacaatgtttaccagtccgaagcccacggcctcccgctgcacctgccagggaacaagtcctcacaccgggaccctgcaccccgaggaccagctcgcttcctgccactaccaggcctgccacccgcacccccggagccacccggaatcctggccccccagccccccgatgtgggctcctcggaccctctgagcatggtgggaccttcccagggccgaagccccagctacgcttcctga

SEQ ID NO: 165 - protein, 209 aa, Artificial Sequence
  Synthetic Construct
MDSDETGFEHSGLWVSVLAGLLLGACQAHPIPDSSPLLQFGGQVRQRYLYTDDAQQTEAHLEIREDGTVGGAADQSPESLLQLKALKPGVIQILGVKTSRFLCQRPDGALYGSLHFDPEACSFRELLLEDGYNVYQSEAHGLPLHLPGNKSSHRDPAPRGPARFLPLPGLPPAPPEPPGILAPQPPDVGSSDPLSMVGPSQGRSPSYAS